European Patent Application EP 4 495 134 A1, published January 22, 2025. Title: Muteinas derivadas de la interleucina-2 humana con actividad superagonista. Applicant: CENTRO DE INMUNOLOGIA MOLECULAR. Application CU 2022-0020, filed March 18, 2022. The sequence listing filed with the application follows.

SEQUENCE LISTING (152 sequences)

SEQ ID NO: 1 - protein, 133 aa, synthetic construct
  VARIANT 81: note = Position 81 is occupied by R, H or K; note (original language) = La posicion 81 esta ocupada por R, H o K
  VARIANT 83: note = Position 83 is occupied by D or E; note (original language) = La posicion 83 esta ocupada por D o E
  VARIANT 84: note = Position 84 is occupied by D or E; note (original language) = La posicion 84 esta ocupada por D o E
  VARIANT 87: note = Position 87 is occupied by D or E; note (original language) = La posicion 87 esta ocupada por D o E
  VARIANT 92: note = Position 92 is occupied by I or L; note (original language) = La posicion 92 esta ocupada por I o L
APTSSSTKKTQLQLEHLLLDLQMILNGINNYKNPKLTRMLTFKFYMPKKATELKHLQCLEEELKPLEEVLNLAQSKNFHLRPRDLISNINVIVLELKGSETTFMCEYADETATIVEFLNRWITFSQSIISTLT

SEQ ID NO: 2 - protein, 133 aa, synthetic construct; identical to SEQ ID NO: 1
  VARIANT 81: note = Position 81 is occupied by D or E; note (original language) = La posicion 81 esta ocupada por D o E
  VARIANT 83: note = Position 83 is occupied by R, H o K; note (original language) = La posicion 81 esta ocupada por R, H o K
  VARIANT 84: note = Position 84 is occupied by D or E; note (original language) = La posicion 84 esta ocupada por D o E
  VARIANT 87: note = Position 87 is occupied by D or E; note (original language) = La posicion 87 esta ocupada por D o E
  VARIANT 92: note = Position 92 is occupied by I or L; note (original language) = La posicion 92 esta ocupada por I o L

SEQ ID NO: 3 - protein, 133 aa, synthetic construct; identical to SEQ ID NO: 1
  VARIANT 81: note = Position 81 is occupied by A, N, G, Q, I, L, M, F, P, S, T, V, W or Y; note (original language) = La posicion 81 esta ocupada por A, N, G, Q, I, L, M, F, P, S, T, V, W o Y
  VARIANT 83: note = Position 83 is occupied by A, N, G, Q, I, L, M, F, P, S, T, V, W or Y; note (original language) = La posicion 83 esta ocupada por A, N, G, Q, I, L, M, F, P, S, T, V, W o Y
  VARIANT 84: note = Positon 84 is occupied by D or E; note (original language) = La posicion 84 esta ocupada por D o E
  VARIANT 87: note = Position 87 is occupied by D or E; note (original language) = La posicion 87 esta ocupada por D o E
  VARIANT 92: note = Position 92 is occupied by I or L; note (original language) = La posicion 92 esta ocupada por I o L

SEQ ID NO: 4 - protein, 133 aa, synthetic construct; identical to SEQ ID NO: 1
  VARIANT 81: note = Position 81 is occupied by D or E; note (original language) = La posicion 81 esta ocupada por D o E
  VARIANT 83: note = Position 83 is occupied by A, N, G, Q, I, L, M, F, P, S, T, V, W or Y; note (original language) = La posicion 83 esta ocupada por A, N, G, Q, I, L, M, F, P, S, T, V, W o Y
  VARIANT 84: note = Position 84 is occupied by D or E; note (original language) = La posicion 84 esta ocupada por D o E
  VARIANT 87: note = Position 87 is occupied by A, N, G, Q, I, L, M, F, P, S, T, V, W or Y; note (original language) = La posición 87 esta ocupada por A, N, G, Q, I, L, M, F, P, S, T, V, W o Y
  VARIANT 92: note = Position 92 is occupied by I or L; note (original language) = La posicion 92 esta ocupada por I o L

SEQ ID NO: 5 - protein, 133 aa, synthetic construct; identical to SEQ ID NO: 1
  VARIANT 81: note = Position 81 is occupied by A, N, G, Q, I, L, M, F, P, S, T, V, W or Y; note (original language) = La posicion 81 esta ocupada por A, N, G, Q, I, L, M, F, P, S, T, V, W o Y
  VARIANT 83: note = Position 83 is occupied by D or E; note (original language) = La posicion 83 esta ocupada por D o E
  VARIANT 84: note = Position 84 is occupied by D or E; note (original language) = La posicion 84 esta ocupada por D o E
  VARIANT 87: note = Position 87 is occupied by A, N, G, Q, I, L, M, F, P, S, T, V, W or Y; note (original language) = La posicion 87 esta ocupada por A, N, G, Q, I, L, M, F, P, S, T, V, W o Y
  VARIANT 92: note = Position 92 is occupied by I or L; note (original language) = La posicion 92 esta ocupada por I o L

SEQ ID NO: 6 - protein, 133 aa, synthetic construct; identical to SEQ ID NO: 1
  VARIANT 81: note = Position 81 is occupied by D or E; note (original language) = La posicion 81 esta ocupada por D o E
  VARIANT 83: note = Position 83 is occupied by D or E; note (original language) = La posicion 83 esta ocupad por D o E
  VARIANT 84: note = Position 84 is occupied by A, N, G, Q, I, L, M, F, P, S, T, V, W or Y; note (original language) = La posicion 84 esta ocupada por A, N, G, Q, I, L, M, F, P, S, T, V, W o Y
  VARIANT 87: note = Position 87 is occupied by A, N, G, Q, I, L, M, F, P, S, T, V, W or Y; note (original language) = La posicion 87 esta coupada por A, N, G, Q, I, L, M, F, P, S, T, V, W o Y
  VARIANT 92: note = Position 92 is occuied by I or L; note (original language) = La posicion 92 esta ocupada por I o L

SEQ ID NO: 7 - protein, 133 aa, synthetic construct; identical to SEQ ID NO: 1
  VARIANT 81: note = Position 81 is occupied by D or E; note (original language) = La posicion 81 esta ocupada por D o E
  VARIANT 83: note = Position 83 is occupied by A, N, G, Q, I, L, M, F, P, S, T, V, W or Y; note (original language) = La posicion 83 esta ocupada por A, N, G, Q, I, L, M, F, P, S, T, V, W o Y
  VARIANT 84: note = Position 84 is occupied by A, N, G, Q, I, L, M, F, P, S, T, V, W or Y; note (original language) = La posicion 84 esta ocupada por A, N, G, Q, I, L, M, F, P, S, T, V, W o Y
  VARIANT 87: note = Position 87 is occupied by D or E; note (original language) = La posicion 87 esta ocupada pro D o E
  VARIANT 92: note = Position 92 is occupied by I or L; note (original language) = La posicion 92 esta ocupada por I o L

SEQ ID NO: 8 - protein, 133 aa, synthetic construct; identical to SEQ ID NO: 1
  VARIANT 81: note = Position 81 is occupied by A, N, G, Q, I, L, M, F, P, S, T, V, W or Y; note (original language) = La posicion 81 esta ocupada por A, N, G, Q, I, L, M, F, P, S, T, V, W o Y
  VARIANT 83: note = Position 83 is occupied by D or E; note (original language) = La posicion 83 esta ocupad por D o E
  VARIANT 84: note = Position 84 is occupied by A, N, G, Q, I, L, M, F, P, S, T, V, W or Y; note (original language) = La posicion 84 esta ocupada por A, N, G, Q, I, L, M, F, P, S, T, V, W o Y
  VARIANT 87: note = Position 87 is occupied by D or E; note (original language) = La posicion 87 esta ocupada por D o E
  VARIANT 92: note = Position 92 is occupied by I or L; note (original language) = La posicion 92 esta ocupada por I o L

SEQ ID NO: 9 - protein, 133 aa, synthetic construct; identical to SEQ ID NO: 1
  VARIANT 81: note = Position 81 is occupied by D or E; note (original language) = La posicion 81 esta ocupada por D o E
  VARIANT 83: note = Position 83 is occupied by A, N, G, Q, I, L, M, F, P, S, T, V, W or Y; note (original language) = La posicion 83 esta ocupada por A, N, G, Q, I, L, M, F, P, S, T, V, W o Y
  VARIANT 84: note = Position 84 is occupied by D or E; note (original language) = La posicion 84 esta ocupada por D or E
  VARIANT 87: note = Position 87 is occupied by D or E; note (original language) = La posicion 87 esta ocupada por D o E
  VARIANT 92: note = Position 92 is occupied by I or L; note (original language) = La posicion 92 esta ocupada por I o L

SEQ ID NO: 10 - protein, 133 aa, synthetic construct; identical to SEQ ID NO: 1
  VARIANT 81: note = Position 81 is occupied by A, N, G, Q, I, L, M, F, P, S, T, V, W or Y; note (original language) = La posicion 81 esta ocupada por A, N, G, Q, I, L, M, F, P, S, T, V, W o Y
  VARIANT 83: note = Position 83 is occupied by D or E; note (original language) = La posicion 83 esta ocupada por D o E
  VARIANT 84: note = Position 84 is occupied by D or E; note (original language) = La posicion 84 esta ocupada por D o E
  VARIANT 87: note = Position 87 is occcupied by D or E; note (original language) = La posicion 87 esta ocupada por D o E
  VARIANT 92: note = Position 92 is occupied by I or L; note (original language) = La posicion 92 esta ocupad por I o L

SEQ ID NO: 11 - protein, 133 aa, synthetic construct; identical to SEQ ID NO: 1
  VARIANT 83: note = Position 83 is occupied by D or E; note (original language) = La posicion 83 esta ocupada por D o E
  VARIANT 84: note = Position 84 is occupied by D or E; note (original language) = La posicion 84 esta ocupada por D o E
  VARIANT 87: note = Position 87 is occupied by A, N, G, Q, I, L, M, F, P, S,T , V, W or Y; note (original language) = La posicion 87 esta ocupada por A, N, G, Q, I, L, M, F, P, S,T , V, W o Y
  VARIANT 92: note = Position 92 is occupied by I or L; note (original language) = La posicion 92 esta ocupada pro I o L
  VARIANT 81: note = Position 81 is occupied by D or E; note (original language) = La posicion 81 esta ocupada por D o E

SEQ ID NO: 12 - protein, 133 aa, synthetic construct; identical to SEQ ID NO: 1
  VARIANT 81: note = Position 81 is occupied by D or E; note (original language) = La posicion 81 esta ocupada por D o E
  VARIANT 83: note = Position 83 is occupied by D or E; note (original language) = La posicion 83 esta ocupada por D o E
  VARIANT 84: note = Positon 84 is occupied by A, N, G, Q, I, L, M, F, P, S, T, V, W or Y; note (original language) = La posicion 84 esta ocupada A, N, G, Q, I, L, M, F, P, S, T, V, W or Y
  VARIANT 87: note = Position 87 is occupied by D or E; note (original language) = La posicion 87 esta ocupada por D o E
  VARIANT 92: note = Position 92 is occupied by I or L; note (original language) = La posicion 92 esta ocupada por I o L

SEQ ID NO: 13 - protein, 133 aa, synthetic construct; identical to SEQ ID NO: 1
  VARIANT 81: note = Position 81 is occupied by D or E; note (original language) = La posicion 81 esta ocupada por D o E
  VARIANT 83: note = Position 83 is occupied by D or E; note (original language) = La posicion 83 esta ocupada por D o E
  VARIANT 84: note = Position 84 is occupied by D or E; note (original language) = La posicion 84 esta ocupada por D o E
  VARIANT 87: note = Position 87 is occupied by D or E; note (original language) = La posicion 87 esta ocupada por D o E
  VARIANT 92: note = Position 92 is occupied by I or L; note (original language) = La posicion 92 esta ocupada por I o L

SEQ ID NO: 14 - protein, 133 aa, synthetic construct; identical to SEQ ID NO: 1
  VARIANT 81: note = Position 81 is occupied by R, H or K; note (original language) = La posicion 81 esta ocupada por R, H o K
  VARIANT 83: note = Position 83 is occupied by D or E; note (original language) = La posicion 83 esta ocupada por D o E
  VARIANT 84: note = Position 84 is occupied by D or E; note (original language) = La posicion 84 está ocupada por D o E
  VARIANT 87: note = Position 87 is occupied by D or E; note (original language) = La posicion 87 esta ocupada por D o E
  VARIANT 92: note = Position 92 is occupied by I or L; note (original language) = La posicion 92 esta ocupada por I o L
  VARIANT 80: note = Position 80 is occupied by F, I, L, M or V; note (original language) = La posicion 80 esta ocupada por F, I, L, M o V
  VARIANT 82: note = Position 82 is occupied by A or P; note (original language) = La posicion 82 esta ocupada por A o P
  VARIANT 85: note = Position 85 is occupied by I, L, M or V; note (original language) = La posicion 85 esta ocupada por I, L, M or V
  VARIANT 86: note = Position 86 is occupied by I or V; note (original language) = La posicion 86 esta ocupada por I o V
  VARIANT 89: note = Position 89 is occupied by I, L or M; note (original language) = La posicion 89 esta ocupada por I, L o M
  VARIANT 93: note = Position 93 is occupied by I, L or V; note (original language) = La posicion 93 esta ocupada por I, L o V

SEQ ID NO: 15 - protein, 133 aa, synthetic construct; identical to SEQ ID NO: 1
  VARIANT 81: note = Position 81 isoccupied by D or E; note (original language) = La posicion 81 esta ocupada por D o E
  VARIANT 83: note = Position 83 is occupied by R, H or K; note (original language) = La posicion 83 esta ocupada por R, H o K
  VARIANT 84: note = Position 84 is occupied by D or E; note (original language) = La posicion 84 esta ocupada por D o E
  VARIANT 87: note = Position 87 is occupied by D or E; note (original language) = La posicion 87 esta ocupada por D o E
  VARIANT 80: note = Position 80 is occupied by F, I, L, M or V; note (original language) = La posicion 80 esta ocupada por F, I, L, M o V
  VARIANT 82: note = Position 82 is occupied by A or P; note (original language) = La posicion 82 esta ocupada por A o P
  VARIANT 85: note = Position 85 is occupied by I, L, M or V; note (original language) = La posicion 85 esta ocupada por I, L, M or V
  VARIANT 86: note = Position 86 is occupied by I or V; note (original language) = La posicion 86 esta ocupada por I o V
  VARIANT 89: note = Position 89 is occupied by I, L or M; note (original language) = La posicion 89 esta ocupada por I, L o M
  VARIANT 93: note = Position 93 is occupied by I, L or V; note (original language) = La posicion 93 esta ocupada por I, L o V
  VARIANT 92: note = Position 92 is occupied by I or L; note (original language) = La posicion 92 esta ocupada por I o L

SEQ ID NO: 16 - protein, 133 aa, synthetic construct; identical to SEQ ID NO: 1
  VARIANT 81: note = Position 81 is occupied by A, N, G, Q, I, L, M, F, P, S, T, V, W or Y; note (original language) = La posicion 81 esta ocupada por A, N, G, Q, I, L, M, F, P, S, T, V, W o Y
  VARIANT 83: note = Position 83 is occupied by A, N, G, Q, I, L, M, F, P, S, T, V, W or Y; note (original language) = La posicion 83 esta ocupada por A, N, G, Q, I, L, M, F, P, S, T, V, W o Y
  VARIANT 84: note = Position 84 is occupied by D or E; note (original language) = La posicion 84 esta ocupada por D o E
  VARIANT 87: note = Position 87 is occupied by D or E; note (original language) = La posicion 87 esta ocupada por D o E
  VARIANT 80: note = Position 80 is occupied by F, I, L, M or V; note (original language) = La posicion 80 esta ocupada por F, I, L, M o V
  VARIANT 82: note = Position 82 is occupied by A or P; note (original language) = La posicion 82 esta ocupada por A o P
  VARIANT 85: note = Position 85 is occupied by I, L, M or V; note (original language) = La posicion 85 esta ocupada por I, L, M or V
  VARIANT 86: note = Position 86 is occupied by I or V; note (original language) = La posicion 86 esta ocupada por I o V
  VARIANT 89: note = Position 89 is occupied by I, L or M; note (original language) = La posicion 89 esta ocupada por I, L o M
  VARIANT 93: note = Position 93 is occupied by I, L or V; note (original language) = La posicion 93 esta ocupada por I, L o V
  VARIANT 92: note = Position 92 is occupied by I or L; note (original language) = La posicion 92 esta ocupada por I o L

SEQ ID NO: 17 - protein, 133 aa, synthetic construct; identical to SEQ ID NO: 1
  VARIANT 81: note = Position 81 is occupied by D or E; note (original language) = La posicion 81 esta ocupada por D o E
  VARIANT 83: note = Position 83 is occupied by A, N, G, Q, I, L, M, F, P, S, T, V, W or Y; note (original language) = La posicion 83 esta ocupada por A, N, G, Q, I, L, M, F, P, S, T, V, W o Y
  VARIANT 84: note = Position 84 is occupied by D or E; note (original language) = La posicion 84 esta ocupada por D o E
  VARIANT 87: note = Position 87 is occupied by A, N, G, Q, I, L, M, F, P, S, T, V, W o Y; note (original language) = La posicion 87 esta ocupada por A, N, G, Q, I, L, M, F, P, S, T, V, W o Y
  VARIANT 80: note = Position 80 is occupied by F, I, L, M or V; note (original language) = La posicion 80 esta ocupada por F, I, L, M o V
  VARIANT 82: note = Position 82 is occupied by A or P; note (original language) = La posicion 82 esta ocupada por A o P
  VARIANT 85: note = Position 85 is occupied by I, L, M or V; note (original language) = La posicion 85 esta ocupada por I, L, M or V
  VARIANT 86: note = Position 86 is occupied by I or V; note (original language) = La posicion 86 esta ocupada por I o V
  VARIANT 89: note = Position 89 is occupied by I, L or M; note (original language) = La posicion 89 esta ocupada por I, L o M
  VARIANT 93: note = Position 93 is occupied by I, L or V; note (original language) = La posicion 93 esta ocupada por I, L o V
  VARIANT 92: note = Position 92 is occupied by I or L; note (original language) = La posicion 92 esta ocupada por I o L

SEQ ID NO: 18 - protein, 133 aa, synthetic construct; identical to SEQ ID NO: 1
  VARIANT 81: note = Position 81 is occupied by A, N, G, Q, I, L, M, F, P, S, T, V, W or Y; note (original language) = La posicion 81 esta ocupada por A, N, G, Q, I, L, M, F, P, S, T, V, W or Y
  VARIANT 83: note = Position 83 is occupied by D or E; note (original language) = La posicion 83 esta ocupada por D o E
  VARIANT 84: note = Position 84 is occupied by D or E; note (original language) = La posicion 84 esta ocupada por D o E
  VARIANT 87: note = Position 87 is occupied by A, N, G, Q, I, L, M, F, P, S, T, V, W or Y; note (original language) = La posocion 87 esta ocupada por A, N, G, Q, I, L, M, F, P, S, T, V, W o Y
  VARIANT 80: note = Position 80 is occupied by F, I, L, M or V; note (original language) = La posicion 80 esta ocupada por F, I, L, M o V
  VARIANT 82: note = Position 82 is occupied by A or P; note (original language) = La posicion 82 esta ocupada por A o P
  VARIANT 85: note = Position 85 is occupied by I, L, M or V; note (original language) = La posicion 85 esta ocupada por I, L, M or V
  VARIANT 86: note = Position 86 is occupied by I or V; note (original language) = La posicion 86 esta ocupada por I o V
  VARIANT 89: note = Position 89 is occupied by I, L or M; note (original language) = La posicion 89 esta ocupada por I, L o M
  VARIANT 93: note = Position 93 is occupied by I, L or V; note (original language) = La posicion 93 esta ocupada por I, L o V
  VARIANT 92: note = Position 92 is occupied by I or L; note (original language) = La posicion 92 esta ocupada por I o L

SEQ ID NO: 19 - protein, 133 aa, synthetic construct; identical to SEQ ID NO: 1
  VARIANT 81: note = Position 81 is occupied by D or E; note (original language) = La posicion 81 esta ocupada por D o E
  VARIANT 83: note = Position 83 is occupied by D or E; note (original language) = La posicion 83 esta ocupada por D o E
  VARIANT 84: note = Position 84 is occupied by A, N, G, Q, I, L, M, F, P, S, T, V, W or Y; note (original language) = La posicion 84 esta ocupada por A, N, G, Q, I, L, M, F, P, S, T, V, W o Y
  VARIANT 87: note = Position 87 is occupied by A, N, G, Q, I, L, M, F, P, S, T, V, W or Y; note (original language) = La posicion 87 esta ocupada por A, N, G, Q, I, L, M, F, P, S, T, V, W o Y
  VARIANT 80: note = Position 80 is occupied by F, I, L, M or V; note (original language) = La posicion 80 esta ocupada por F, I, L, M o V
  VARIANT 82: note = Position 82 is occupied by A or P; note (original language) = La posicion 82 esta ocupada por A o P
  VARIANT 85: note = Position 85 is occupied by I, L, M or V; note (original language) = La posicion 85 esta ocupada por I, L, M or V
  VARIANT 86: note = Position 86 is occupied by I or V; note (original language) = La posicion 86 esta ocupada por I o V
  VARIANT 89: note = Position 89 is occupied by I, L or M; note (original language) = La posicion 89 esta ocupada por I, L o M
  VARIANT 93: note = Position 93 is occupied by I, L or V; note (original language) = La posicion 93 esta ocupada por I, L o V
  VARIANT 92: note = Position 92 is occupied by I or L; note (original language) = La posicion 92 esta ocupada por I o L

SEQ ID NO: 20 - protein, 133 aa, synthetic construct; identical to SEQ ID NO: 1
  VARIANT 81: note = Position 81 is occupied by D or E; note (original language) = La posicion 81 esta ocupada por D o E
  VARIANT 83: note = Position 83 is occupied by A, N, G, Q, I, L, M, F, P, S, T, V, W or Y; note (original language) = La posicion 83 esta ocupada por A, N, G, Q, I, L, M, F, P, S, T, V, W or Y
  VARIANT 84: note = Position 84 is occupied by A, N, G, Q, I, L, M, F, P, S, T, V, W or Y; note (original language) = La posicion 84 esta ocupada por A, N, G, Q, I, L, M, F, P, S, T, V, W or Y
  VARIANT 87: note = Position 87 is occupied by D or E; note (original language) = La posicion 87 esta ocupada por D o E
  VARIANT 80: note = Position 80 is occupied by F, I, L, M or V; note (original language) = La posicion 80 esta ocupada por F, I, L, M o V
  VARIANT 82: note = Position 82 is occupied by A or P; note (original language) = La posicion 82 esta ocupada por A o P
  VARIANT 85: note = Position 85 is occupied by I, L, M or V; note (original language) = La posicion 85 esta ocupada por I, L, M or V
  VARIANT 86: note = Position 86 is occupied by I or V; note (original language) = La posicion 86 esta ocupada por I o V
  VARIANT 89: note = Position 89 is occupied by I, L or M; note (original language) = La posicion 89 esta ocupada por I, L o M
  VARIANT 93: note = Position 93 is occupied by I, L or V; note (original language) = La posicion 93 esta ocupada por I, L o V
  VARIANT 92: note = Position 92 is occupied by I or L; note (original language) = La posicion 92 esta ocupada por I o L

SEQ ID NO: 21 - protein, 133 aa, synthetic construct; identical to SEQ ID NO: 1
  VARIANT 81: note = Position 81 is occupied by A, N, G, Q, I, L, M, F, P, S, T, V, W or Y; note (original language) = La posicion 81 esta ocupada A, N, G, Q, I, L, M, F, P, S, T, V, W o Y
  VARIANT 83: note = Position 83 is occupied by D or E; note (original language) = La posicin 83 esta ocupada por D o E
  VARIANT 84: note = Position 84 is occupied by A, N, G, Q, I, L, M, F, P, S, T, V, W or Y; note (original language) = La posicion 84 esta ocupada por A, N, G, Q, I, L, M, F, P, S, T, V, W o Y
  VARIANT 87: note = Position 87 is occupied by D or E; note (original language) = La posicion 87 esta ocupada por D o E
  VARIANT 80: note = Position 80 is occupied by F, I, L, M or V; note (original language) = La posicion 80 esta ocupada por F, I, L, M o V
  VARIANT 82: note = Position 82 is occupied by A or P; note (original language) = La posicion 82 esta ocupada por A o P
  VARIANT 85: note = Position 85 is occupied by I, L, M or V; note (original language) = La posicion 85 esta ocupada por I, L, M or V
  VARIANT 86: note = Position 86 is occupied by I or V; note (original language) = La posicion 86 esta ocupada por I o V
  VARIANT 89: note = Position 89 is occupied by I, L or M; note (original language) = La posicion 89 esta ocupada por I, L o M
  VARIANT 93: note = Position 93 is occupied by I, L or V; note (original language) = La posicion 93 esta ocupada por I, L o V
  VARIANT 92: note = Position 92 is occupied by I or L; note (original language) = La posicion 92 esta ocupada por I o L

SEQ ID NO: 22 - protein, 133 aa, synthetic construct; identical to SEQ ID NO: 1
  VARIANT 81: note = Position 81 is occupied by D or E; note (original language) = La posicion 81 esta ocupada por D o E
  VARIANT 83: note = Position 83 is occupied by A, N, G, Q, I, L, M, F, P, S, T, V, W or Y; note (original language) = La posicion 83 esta ocupada por A, N, G, Q, I, L, M, F, P, S, T, V, W o Y
  VARIANT 84: note = Position 84 is occupoed by D or E; note (original language) = La posicion 84 esta ocupada por D o E
  VARIANT 87: note = Position 87 is occupied by D or E; note (original language) = La posicion 87 esta ocupada por D o E
  VARIANT 80: note = Position 80 is occupied by F, I, L, M or V; note (original language) = La posicion 80 esta ocupada por F, I, L, M o V
  VARIANT 82: note = Position 82 is occupied by A or P; note (original language) = La posicion 82 esta ocupada por A o P
  VARIANT 85: note = Position 85 is occupied by I, L, M or V; note (original language) = La posicion 85 esta ocupada por I, L, M or V
  VARIANT 86: note = Position 86 is occupied by I or V; note (original language) = La posicion 86 esta ocupada por I o V
  VARIANT 89: note = Position 89 is occupied by I, L or M; note (original language) = La posicion 89 esta ocupada por I, L o M
  VARIANT 93: note = Position 93 is occupied by I, L or V; note (original language) = La posicion 93 esta ocupada por I, L o V
  VARIANT 92: note = Position 92 is occupied by I or L; note (original language) = La posicion 92 esta ocupada por I o L

SEQ ID NO: 23 - protein, 133 aa, synthetic construct; identical to SEQ ID NO: 1
  VARIANT 81: note = Position 81 is occupied by A, N, G, Q, I, L, M, F, P, S, T, V, W or Y; note (original language) = La posicion 81 esta ocupada por A, N, G, Q, I, L, M, F, P, S, T, V, W o Y
  VARIANT 83: note = Position 83 is occupied by D or E; note (original language) = La posicion 83 esta ocupada por D o E
  VARIANT 84: note = Position 84 is occupied by D or E; note (original language) = La posocion 84 esta ocupada por D o E
  VARIANT 87: note = Position 87 is occupied by D or E; note (original language) = La posicion esta ocupada por D o E
  VARIANT 80: note = Position 80 is occupied by F, I, L, M or V; note (original language) = La posicion 80 esta ocupada por F, I, L, M o V
  VARIANT 82: note = Position 82 is occupied by A or P; note (original language) = La posicion 82 esta ocupada por A o P
  VARIANT 85: note = Position 85 is occupied by I, L, M or V; note (original language) = La posicion 85 esta ocupada por I, L, M or V
  VARIANT 86: note = Position 86 is occupied by I or V; note (original language) = La posicion 86 esta ocupada por I o V
  VARIANT 89: note = Position 89 is occupied by I, L or M; note (original language) = La posicion 89 esta ocupada por I, L o M
  VARIANT 93: note = Position 93 is occupied by I, L or V; note (original language) = La posicion 93 esta ocupada por I, L o V
  VARIANT 92: note = Position 92 is occupied by I or L; note (original language) = La posicion 92 esta ocupada por I o L

SEQ ID NO: 24 - protein, 133 aa, synthetic construct; identical to SEQ ID NO: 1
  VARIANT 83: note = Position 83 is occupied by D or E; note (original language) = La posicion 83 esta ocupada por D o E
  VARIANT 84: note = Position 84 is occupied by D or E; note (original language) = La posicion 84 esta ocupada por D o E
  VARIANT 87: note = Position 87 is occupied by A, N, G, Q, I, L, M, F, P, S, T, V, W or Y; note (original language) = La posicion 87 esta ocupada por A, N, G, Q, I, L, M, F, P, S, T, V, W o Y
  VARIANT 81: note = Position 81 is occupied by D or E; note (original language) = La posicin 81 esta ocupada por D o E
  VARIANT 80: note = Position 80 is occupied by F, I, L, M or V; note (original language) = La posicion 80 esta ocupada por F, I, L, M o V
  VARIANT 82: note = Position 82 is occupied by A or P; note (original language) = La posicion 82 esta ocupada por A o P
  VARIANT 85: note = Position 85 is occupied by I, L, M or V; note (original language) = La posicion 85 esta ocupada por I, L, M or V
  VARIANT 86: note = Position 86 is occupied by I or V; note (original language) = La posicion 86 esta ocupada por I o V
  VARIANT 89: note = Position 89 is occupied by I, L or M; note (original language) = La posicion 89 esta ocupada por I, L o M
  VARIANT 93: note = Position 93 is occupied by I, L or V; note (original language) = La posicion 93 esta ocupada por I, L o V
  VARIANT 92: note = Position 92 is occupied by I or L; note (original language) = La posicion 92 esta ocupada por I o L

SEQ ID NO: 25 - protein, 133 aa, synthetic construct; identical to SEQ ID NO: 1
  VARIANT 81: note = Position 81 is occupied by D or E; note (original language) = La posicion 81 esta ocupada por D o E
  VARIANT 83: note = Position 83 is occupied by D or E; note (original language) = La posicion 83 esta ocupada por D o E
  VARIANT 84: note = Position 84 is occupied by A, N, G, Q, I, L, M, F, P, S, T, V, W or Y; note (original language) = La posicion 84 esta ocupada por A, N, G, Q, I, L, M, F, P, S, T, V, W o Y
  VARIANT 87: note = Position 87 is occupied by D or E; note (original language) = La posicion 87 esta ocupada por D o E
  VARIANT 80: note = Position 80 is occupied by F, I, L, M or V; note (original language) = La posicion 80 esta ocupada por F, I, L, M o V
  VARIANT 82: note = Position 82 is occupied by A or P; note (original language) = La posicion 82 esta ocupada por A o P
  VARIANT 85: note = Position 85 is occupied by I, L, M or V; note (original language) = La posicion 85 esta ocupada por I, L, M or V
  VARIANT 86: note = Position 86 is occupied by I or V; note (original language) = La posicion 86 esta ocupada por I o V
  VARIANT 89: note = Position 89 is occupied by I, L or M; note (original language) = La posicion 89 esta ocupada por I, L o M
  VARIANT 93: note = Position 93 is occupied by I, L or V; note (original language) = La posicion 93 esta ocupada por I, L o V
  VARIANT 92: note = Position 92 is occupied by I or L; note (original language) = La posicion 92 esta ocupada por I o L

SEQ ID NO: 26 - protein, 133 aa, synthetic construct; identical to SEQ ID NO: 1
  VARIANT 81: note = Position 81 is occupied by D or E; note (original language) = La poisicoin 81 esta ocupada por D o E
  VARIANT 83: note = Position 83 is occupied by D or E; note (original language) = La posicion 83 esta ocupada por D o E
  VARIANT 84: note = Position 84 is occupied by D or E; note (original language) = L aposicion 84 esta ocupada por D o E
  VARIANT 87: note = Position 87 is occupied by D or E; note (original language) = La posicion 87 esta ocupad por D o E
  VARIANT 80: note = Position 80 is occupied by F, I, L, M or V; note (original language) = La posicion 80 esta ocupada por F, I, L, M o V
  VARIANT 82: note = Position 82 is occupied by A or P; note (original language) = La posicion 82 esta ocupada por A o P
  VARIANT 85: note = Position 85 is occupied by I, L, M or V; note (original language) = La posicion 85 esta ocupada por I, L, M or V
  VARIANT 86: note = Position 86 is occupied by I or V; note (original language) = La posicion 86 esta ocupada por I o V
  VARIANT 89: note = Position 89 is occupied by I, L or M; note (original language) = La posicion 89 esta ocupada por I, L o M
  VARIANT 93: note = Position 93 is occupied by I, L or V; note (original language) = La posicion 93 esta ocupada por I, L o V
  VARIANT 92: note = Position 92 is occupied by I or L; note (original language) = La posicion 92 esta ocupada por I o L

SEQ ID NO: 27 - protein, 133 aa, synthetic construct
  VARIANT 81: note = Position 81 is occupied by H,K or R; note (original language) = La posicion 80 esta ocupada por H,K o R
  VARIANT 83: note = Position 83 is occupied by D or E; note (original language) = La posicion 83 esta ocupada por D o E
  VARIANT 84: note = Position 84 is occupied by D or E; note (original language) = La posicion 84 esta ocupada por D o E
  VARIANT 87: note = Position 87 is occupied by D or E; note (original language) = La posicion 87 esta ocupada por D o E
  VARIANT 92: note = Position 92 is occupied by I or L; note (original language) = La posicion 92 esta ocupada por I o L
  VARIANT 35: note = Position 35 is occupied by D, E or Q; note (original language) = La posicion 35 esta ocupada por D, E o Q
APTSSSTKKTQLQLEHLLLDLQMILNGINNYKNPKLTAMLTAKFAMPKKATELKHLQCLEEEAKPLEEVLNLAQSKNFHLRPRDLISNINVIVLELKGSETTFMCEYADETATIVEFLNRWITFSQSIISTLT

SEQ ID NO: 28 - protein, 133 aa, synthetic construct; identical to SEQ ID NO: 1
  VARIANT 81: note = Position 81 is occupied by D or E; note (original language) = La posicion 81 esta ocupada por D o E
  VARIANT 83: note = Position 83 is occupied by H,K or R; note (original language) = La posicion 83 esta ocupada por H,K o R
  VARIANT 84: note = Position 84 is occupied by D or E; note (original language) = La posicion 84 esta ocupada por D o E
  VARIANT 87: note = Position 87 is occupied by D or E; note (original language) = La posicion 87 esta ocupada por D o E
  VARIANT 92: note = Position 92 is occupied by I or L; note (original language) = La posicion 92 esta ocupada por I o L
  VARIANT 35: note = Position 35 is occupied by D, E or Q; note (original language) = La posicion 35 esta ocupada por D, E o Q

SEQ ID NO: 29 - protein, 133 aa, synthetic construct; identical to SEQ ID NO: 1
  VARIANT 81: note = Position 81 is occupied by A, N, G, Q, I, L, M, F, P, S, T, V, W or Y; note (original language) = La posicion 81 esta ocupada por A, N, G, Q, I, L, M, F, P, S, T, V, W o Y
  VARIANT 83: note = Position 83 is occupied by A, N, G, Q, I, L, M, F, P, S, T, V, W or Y; note (original language) = La posicion 83 esta ocupada por A, N, G, Q, I, L, M, F, P, S, T, V, W o Y
  VARIANT 84: note = Position 84 is occupied by D or E; note (original language) = La posicion 84 esta ocupada por D o E
  VARIANT 87: note = Position 87 is occupied by D or E; note (original language) = La posicion 87 esta ocupada por D o E
  VARIANT 92: note = Position 92 is occupied by I or L; note (original language) = La posicion 92 esta ocupada por I o L
  VARIANT 35: note = Position 35 is occupied by D, E or Q; note (original language) = La posicion 35 esta ocupada por D, E o Q

SEQ ID NO: 30 - protein, 133 aa, synthetic construct; identical to SEQ ID NO: 1
  VARIANT 81: note = Position 81 is occupied by D or E; note (original language) = La posicion 81 esta ocupada por D o E
  VARIANT 83: note = Position 83 is occupied by A, N, G, Q, I, L, M, F, P, S, T, V, W or Y; note (original language) = La posicion 83 esta ocupada por A, N, G, Q, I, L, M, F, P, S, T, V, W o Y
  VARIANT 84: note = Position 84 is occupied by D or E; note (original language) = La posicion 84 esta ocupada por D o E
  VARIANT 87: note = Position 87 is occupied by A, N, G, Q, I, L, M, F, P, S, T, V, W or Y; note (original language) = La posicion 87 esta ocupada por A, N, G, Q, I, L, M, F, P, S, T, V, W o Y
  VARIANT 92: note = Position 92 is occupied by I or L; note (original language) = La posicion 92 esta ocupada por I o L
  VARIANT 35: note = Position 35 is occupied by D, E or Q; note (original language) = La posicion 35 esta ocupada por D, E o Q

SEQ ID NO: 31 - protein, 133 aa, synthetic construct; identical to SEQ ID NO: 1
  VARIANT 81: note = Position 81 is occupied by A, N, G, Q, I, L, M, F, P, S, T, V, W or Y; note (original language) = La posicion 81 esta ocupada por A, N, G, Q, I, L, M, F, P, S, T, V, W o Y
  VARIANT 83: note = Position 83 is occupied by D or E; note (original language) = La posicion 83 esta ocupada por D o E
  VARIANT 84: note = Position 84 is occupied by D or E; note (original language) = La posicion 84 esta ocupada por D o E
  VARIANT 87: note = Position 87 is occupied by A, N, G, Q, I, L, M, F, P, S, T, V, W or Y; note (original language) = La posicion 87 esta ocupada por A, N, G, Q, I, L, M, F, P, S, T, V, W o Y
  VARIANT 92: note = Position 92 is occupied by I or L; note (original language) = La posicion 92 esta ocupada por I o L
  VARIANT 35: note = Position 35 is occupied by D, E or Q; note (original language) = La posicion 35 esta ocupada por D, E o Q

SEQ ID NO: 32 - protein, 133 aa, synthetic construct; identical to SEQ ID NO: 1
  VARIANT 81: note = Position 81 is occupied by D or E; note (original language) = La posicion 81 esta ocupada por D o E
  VARIANT 83: note = Position 83 is occupied by D or E; note (original language) = La posicion 83 esta ocupada por D o E
  VARIANT 84: note = Position 84 is occupied by A, N, G, Q, I, L, M, F, P, S, T, V, W or Y; note (original language) = La posicion 84 esta ocupada por A, N, G, Q, I, L, M, F, P, S, T, V, W o Y
  VARIANT 87: note = Position 87 is occupied by A, N, G, Q, I, L, M, F, P, S, T, V, W or Y; note (original language) = La posicion 87 esta ocupada por A, N, G, Q, I, L, M, F, P, S, T, V, W o Y
  VARIANT 92: note = Position 92 is occupied by I or L; note (original language) = La posicion 92 esta ocupada por I o L
  VARIANT 35: note = Position 35 is occupied by D, E or Q; note (original language) = La posicion 35 esta ocupada por D, E o Q

SEQ ID NO: 33 - protein, 133 aa, synthetic construct; identical to SEQ ID NO: 1
  VARIANT 81: note = Position 81 is occupied by D or E; note (original language) = La posicion 81 esta ocupada por D o E
  VARIANT 83: note = Position 83 is occupied by A, N, G, Q, I, L, M, F, P, S, T, V, W or Y; note (original language) = La posicion 83 esta ocupada por A, N, G, Q, I, L, M, F, P, S, T, V, W o Y
  VARIANT 84: note = Position 84 is occupied by A, N, G, Q, I, L, M, F, P, S, T, V, W or Y; note (original language) = La posicion 84 esta ocupada por A, N, G, Q, I, L, M, F, P, S, T, V, W o Y
  VARIANT 87: note = Position 87 is occupied by D or E; note (original language) = La posicion 87 esta ocupada por D o E
  VARIANT 92: note = Position 92 is occupied by I or L; note (original language) = La posicion 92 esta ocupada por I o L
  VARIANT 35: note = Position 35 is occupied by D, E or Q; note (original language) = La posicion 35 esta ocupada por D, E o Q

SEQ ID NO: 34 - protein, 133 aa, synthetic construct; identical to SEQ ID NO: 1
  VARIANT 81: note = Position 81 is occupied by A, N, G, Q, I, L, M, F, P, S, T, V, W or Y; note (original language) = La posicion 81 esta ocupada por A, N, G, Q, I, L, M, F, P, S, T, V, W o Y
  VARIANT 83: note = Position 83 is occupied by D or E; note (original language) = La posicion 83 esta ocupada por D o E
  VARIANT 84: note = Position 84 is occupied by A, N, G, Q, I, L, M, F, P, S, T, V, W or Y; note (original language) = La posicion 84 esta ocupada por A, N, G, Q, I, L, M, F, P, S, T, V, W o Y
  VARIANT 87: note = Position 87 is occupied by D or E; note (original language) = La posicion 87 esta ocupada por D o E
  VARIANT 92: note = Position 92 is occupied by I or L; note (original language) = La posicion 92 esta ocupada por I o L
  VARIANT 35: note = Position 35 is occupied by D, E or Q; note (original language) = La posicion 35 esta ocupada por D, E o Q

SEQ ID NO: 35 - protein, 133 aa, synthetic construct; identical to SEQ ID NO: 1
  VARIANT 81: note = Position 81 is occupied by D or E; note (original language) = La posicion 81 esta ocupada por D o E
  VARIANT 83: note = Position 83 is occupied by A, N, G, Q, I, L, M, F, P, S, T, V, W or Y; note (original language) = La posicion 83 esta ocupada por A, N, G, Q, I, L, M, F, P, S, T, V, W o Y
  VARIANT 84: note = Position 84 is occupied by D or E; note (original language) = La posicion 84 esta ocupada por D o E
  VARIANT 87: note = Position 87 is occupied by D or E; note (original language) = La posicion 87 esta ocupada por D o E
  VARIANT 92: note = Position 92 is occupied by I or L; note (original language) = La posicion 92 esta ocupada por I o L
  VARIANT 35: note = Position 35 is occupied by D, E or Q; note (original language) = La posicion 35 esta ocupada por D, E o Q

SEQ ID NO: 36 - protein, 133 aa, synthetic construct; identical to SEQ ID NO: 1
  VARIANT 81: note = Position 81 is occupied by A, N, G, Q, I, L, M, F, P, S, T, V, W or Y; note (original language) = La posicion 81 esta ocupada por A, N, G, Q, I, L, M, F, P, S, T, V, W o Y
  VARIANT 83: note = Position 83 is occupied by D or E; note (original language) = La posicion 83 esta ocupada por D o E
  VARIANT 84: note = Position 84 is occupied by D or E; note (original language) = La posicion 84 esta ocupada por D o E
  VARIANT 87: note = Position 87 is occupied by D or E; note (original language) = La posicion 87 esta ocupada por D o E
  VARIANT 92: note = Position 92 is occupied by I or L; note (original language) = La posicion 92 esta ocupada por I o L
  VARIANT 35: note = Position 35 is occupied by D, E or Q; note (original language) = La posicion 35 esta ocupada por D, E o Q
  VARIANT 35: note = Position 35 is occupied by D, E or Q; note (original language) = La posicion 35 esta ocupada por D, E o Q

SEQ ID NO: 37 - protein, 133 aa, synthetic construct; identical to SEQ ID NO: 1
  VARIANT 81: note = Position 81 is occupied by D or E; note (original language) = La posicion 81 esta ocupada por D o E
  VARIANT 83: note = Position 83 is occupied by D or E; note (original language) = La posicion 83 esta ocupada por D o E
  VARIANT 84: note = Position 84 is occupied by D or E; note (original language) = La posicion 84 esta ocupada por D o E
  VARIANT 87: note = Position 87 is occupied by A, N, G, Q, I, L, M, F, P, S, T, V, W or Y; note (original language) = La posicion 87 esta ocupada por A, N, G, Q, I, L, M, F, P, S, T, V, W o Y
  VARIANT 92: note = Position 92 is occupied by I or L; note (original language) = La posicion 92 esta ocupada por I o L
  VARIANT 35: note = Position 35 is occupied by D, E or Q; note (original language) = La posicion 35 esta ocupada por D, E o Q

SEQ ID NO: 38 - protein, 133 aa, synthetic construct; identical to SEQ ID NO: 1
  VARIANT 81: note = Position 81 is occupied by D or E; note (original language) = La posicion 81 esta ocupada por D o E
  VARIANT 83: note = Position 83 is occupied by D or E; note (original language) = La posicion 83 esta ocupada por D o E
  VARIANT 84: note = Position 84 is occupied by A, N, G, Q, I, L, M, F, P, S, T, V, W or Y; note (original language) = La posicion 84 esta ocupada por A, N, G, Q, I, L, M, F, P, S, T, V, W o Y
  VARIANT 87: note = Position 87 is occupied by D or E; note (original language) = La posicion 87 esta ocupada por D o E
  VARIANT 92: note = Position 92 is occupied by I or L; note (original language) = La posicion 92 esta ocupada por I o L
  VARIANT 35: note = Position 35 is occupied by D, E or Q; note (original language) = La posicion 35 esta ocupada por D, E o Q

SEQ ID NO: 39 - protein, 133 aa, synthetic construct; identical to SEQ ID NO: 1
  VARIANT 81: note = Position 81 is occupied by D or E; note (original language) = La posicion 81 esta ocupada por D o E
  VARIANT 83: note = Position 83 is occupied by D or E; note (original language) = La posicion 83 esta ocupada por D o E
  VARIANT 84: note = Position 84 is occupied by D or E; note (original language) = La posicion 84 esta ocupada por D o E
  VARIANT 87: note = Position 84 is occupied by D or E; note (original language) = La posicion 84 esta ocupada por D o E
  VARIANT 92: note = Position 92 is occupied by I or L; note (original language) = La posicion 92 esta ocupada por I o L
  VARIANT 35: note = Position 35 is occupied by D, E or Q; note (original language) = La posicion 35 esta ocupada por D, E o Q
  VARIANT 87: note = Position 87 is occupied by D or E; note (original language) = La posicion 87 esta ocupada por D o E

SEQ ID NO: 40 - protein, 133 aa, synthetic construct; identical to SEQ ID NO: 1
  VARIANT 81: note = Position 81 is occupied by H,K or R; note (original language) = La posicion 81 esta ocupada por H,K o R
  VARIANT 83: note = Position 83 is occupied by D or E; note (original language) = La posicion 83 esta ocupada por D o E
  VARIANT 84: note = Position 84 is occupied by D or E; note (original language) = La posicion 84 esta ocupada por D o E
  VARIANT 87: note = Position 87 is occupied by D or E; note (original language) = La posicion 87 esta ocupada por D o E
  VARIANT 80: note = Position 80 is occupied by L, F, M, V or I; note (original language) = La posicion 80 esta ocupada por L, F, M, V o I
  VARIANT 82: note = Position 82 is occupied by P or A; note (original language) = La posicion 82 esta ocupada por P o A
  VARIANT 85: note = Position 85 is occupied by L. I, V or M; note (original language) = La posicion 85 esta ocupada por L, I, V, M
  VARIANT 86: note = Position 86 is occupied by I or V; note (original language) = La posicion 86 esta ocupada por I o V
  VARIANT 89: note = Position 89 is occupied by I, L or M; note (original language) = La posicion 89 esta ocupada por I, L o M
  VARIANT 92: note = Position 92 is occupied by I or L; note (original language) = La posicion 92 esta ocupada por I o L
  VARIANT 93: note = Position 93 is occupied by I, L or V; note (original language) = La posicion 93 esta ocupada por I, L o V
  VARIANT 35: note = Position 35 is occupied by D, E or Q; note (original language) = La posicion 35 esta ocupada por D, E o Q

SEQ ID NO: 41 - protein, 133 aa, synthetic construct; identical to SEQ ID NO: 1
  VARIANT 81: note = Position 81 is occupied by D or E; note (original language) = La posicion 81 esta ocupada por D o E
  VARIANT 83: note = Position 83 is occupied by H,K or R; note (original language) = La posicion 83 esta ocupada por H,K o R
  VARIANT 84: note = Position 84 is occupied by D or E; note (original language) = La posicion 84 esta ocupada por D o E
  VARIANT 87: note = Position 87 is occupied by D or E; note (original language) = La posicion 87 esta ocupada por D o E
  VARIANT 80: note = Position 80 is occupied by F, I, L, M or V; note (original language) = La posicion 80 esta ocupada por F, I, L, M o V
  VARIANT 82: note = Position 82 is occupied by A or P; note (original language) = La posicion 82 esta ocupada por A o P
  VARIANT 85: note = Position 85 is occupied by I, L, M or V; note (original language) = La posicion 85 esta ocupada por I, L, M or V
  VARIANT 86: note = Position 86 is occupied by I or V; note (original language) = La posicion 86 esta ocupada por I o V
  VARIANT 89: note = Position 89 is occupied by I, L or M; note (original language) = La posicion 89 esta ocupada por I, L o M
  VARIANT 92: note = Position 92 is occupied by I or L; note (original language) = La posicion 92 esta ocupada por I o L
  VARIANT 93: note = Position 93 is occupied by I, L or V; note (original language) = La posicion 93 esta ocupada por I, L o V
  VARIANT 35: note = Position 35 is occupied by D, E or Q; note (original language) = La posicion 35 esta ocupada por D, E o Q

SEQ ID NO: 42 - protein, 133 aa, synthetic construct; identical to SEQ ID NO: 1
  VARIANT 81: note = Position 81 is occupied by A, N, G, Q, I, L, M, F, P, S, T, V, W or Y; note (original language) = La posicion 81 esta ocupada por A, N, G, Q, I, L, M, F, P, S, T, V, W o Y
  VARIANT 83: note = Position 83 is occupied by A, N, G, Q, I, L, M, F, P, S, T, V, W or Y; note (original language) = La posicion 83 esta ocupada por A, N, G, Q, I, L, M, F, P, S, T, V, W o Y
  VARIANT 84: note = Position 84 is occupied by D or E; note (original language) = La posicion 84 esta ocupada por D o E
  VARIANT 87: note = Position 87 is occupied by D or E; note (original language) = La posicion 87 esta ocupada por D o E
  VARIANT 80: note = Position 80 is occupied by F, I, L, M or V; note (original language) = La posicion 80 esta ocupada por F, I, L, M o V
  VARIANT 82: note = Position 82 is occupied by A or P; note (original language) = La posicion 82 esta ocupada por A o P
  VARIANT 85: note = Position 85 is occupied by I, L, M or V; note (original language) = La posicion 85 esta ocupada por I, L, M or V
  VARIANT 86: note = Position 86 is occupied by I or V; note (original language) = La posicion 86 esta ocupada por I o V
  VARIANT 89: note = Position 89 is occupied by I, L or M; note (original language) = La posicion 89 esta ocupada por I, L o M
  VARIANT 92: note = Position 92 is occupied by I or L; note (original language) = La posicion 92 esta ocupada por I o L
  VARIANT 93: note = Position 93 is occupied by I, L or V; note (original language) = La posicion 93 esta ocupada por I, L o V
  VARIANT 35: note = Position 35 is occupied by D, E or Q; note (original language) = La posicion 35 esta ocupada por D, E o Q

SEQ ID NO: 43 - protein, 133 aa, synthetic construct; identical to SEQ ID NO: 1
  VARIANT 81: note = Position 81 is occupied by D or E; note (original language) = La posicion 81 esta ocupada por D o E; note = Position 81 is occupied by D or E; note (original language) = La posicion 81 esta ocupada por D o E
  VARIANT 83: note = Position 83 is occupied by A, N, G, Q, I, L, M, F, P, S, T, V, W or Y; note (original language) = La posicion 83 esta ocupada por A, N, G, Q, I, L, M, F, P, S, T, V, W o Y
  VARIANT 84: note = Position 84 is occupied by D or E; note (original language) = La posicion 84 esta ocupada por D o E
  VARIANT 87: note = Position 87 is occupied by A, N, G, Q, I, L, M, F, P, S, T, V, W or Y; note (original language) = La posicion 87 esta ocupada por A, N, G, Q, I, L, M, F, P, S, T, V, W o Y
  VARIANT 80: note = Position 80 is occupied by F, I, L, M or V; note (original language) = La posicion 80 esta ocupada por F, I, L, M o V
  VARIANT 82: note = Position 82 is occupied by A or P; note (original language) = La posicion 82 esta ocupada por A o P
  VARIANT 85: note = Position 85 is occupied by I, L, M or V; note (original language) = La posicion 85 esta ocupada por I, L, M or V
  VARIANT 86: note = Position 86 is occupied by I or V; note (original language) = La posicion 86 esta ocupada por I o V
  VARIANT 89: note = Position 89 is occupied by I, L or M; note (original language) = La posicion 89 esta ocupada por I, L o M
  VARIANT 92: note = Position 92 is occupied by I or L; note (original language) = La posicion 92 esta ocupada por I o L
  VARIANT 93: note = Position 93 is occupied by I, L or V; note (original language) = La posicion 93 esta ocupada por I, L o V
  VARIANT 35: note = Position 35 is occupied by D, E or Q; note (original language) = La posicion 35 esta ocupada por D, E o Q

SEQ ID NO: 44 - protein, 133 aa, synthetic construct; identical to SEQ ID NO: 1
  VARIANT 81: note = Position 81 is occupied by A, N, G, Q, I, L, M, F, P, S, T, V, W or Y; note (original language) = La posicion 81 esta ocupada por A, N, G, Q, I, L, M, F, P, S, T, V, W o Y
  VARIANT 83: note = Position 83 is occupied by D or E; note (original language) = La posicion 83 esta ocupada por D o E
  VARIANT 84: note = Position 84 is occupied by D or E; note (original language) = La posicion 84 esta ocupada por D o E
  VARIANT 87: note = Position 87 is occupied by A, N, G, Q, I, L, M, F, P, S, T, V, W or Y; note (original language) = La posicion 81 esta ocupada por A, N, G, Q, I, L, M, F, P, S, T, V, W o Y
  VARIANT 80: note = Position 80 is occupied by F, I, L, M or V; note (original language) = La posicion 80 esta ocupada por F, I, L, M o V
  VARIANT 82: note = Position 82 is occupied by A or P; note (original language) = La posicion 82 esta ocupada por A o P
  VARIANT 85: note = Position 85 is occupied by I, L, M or V; note (original language) = La posicion 85 esta ocupada por I, L, M or V
  VARIANT 86: note = Position 86 is occupied by I or V; note (original language) = La posicion 86 esta ocupada por I o V
  VARIANT 89: note = Position 89 is occupied by I, L or M; note (original language) = La posicion 89 esta ocupada por I, L o M
  VARIANT 92: note = Position 92 is occupied by I or L; note (original language) = La posicion 92 esta ocupada por I o L
  VARIANT 93: note = Position 93 is occupied by I, L or V; note (original language) = La posicion 93 esta ocupada por I, L o V
  VARIANT 35: note = Position 35 is occupied by D, E or Q; note (original language) = La posicion 35 esta ocupada por D, E o Q

SEQ ID NO: 45 - protein, 133 aa, synthetic construct; identical to SEQ ID NO: 1
  VARIANT 81: note = Position 81 is occupied by D or E; note (original language) = La posicion 81 esta ocupada por D o E
  VARIANT 83: note = Position 83 is occupied by D or E; note (original language) = La posicion 83 esta ocupada por D o E
  VARIANT 84: note = Position 84 is occupied by A, N, G, Q, I, L, M, F, P, S, T, V, W or Y; note (original language) = La posicion 84 esta ocupada por A, N, G, Q, I, L, M, F, P, S, T, V, W o Y
  VARIANT 87: note = Position 87 is occupied by A, N, G, Q, I, L, M, F, P, S, T, V, W or Y; note (original language) = La posicion 87 esta ocupada por A, N, G, Q, I, L, M, F, P, S, T, V, W o Y
  VARIANT 80: note = Position 80 is occupied by F, I, L, M or V; note (original language) = La posicion 80 esta ocupada por F, I, L, M o V
  VARIANT 82: note = Position 82 is occupied by A or P; note (original language) = La posicion 82 esta ocupada por A o P
  VARIANT 85: note = Position 85 is occupied by I, L, M or V; note (original language) = La posicion 85 esta ocupada por I, L, M or V
  VARIANT 86: note = Position 86 is occupied by I or V; note (original language) = La posicion 86 esta ocupada por I o V
  VARIANT 89: note = Position 89 is occupied by I, L or M; note (original language) = La posicion 89 esta ocupada por I, L o M
  VARIANT 92: note = Position 92 is occupied by I or L; note (original language) = La posicion 92 esta ocupada por I o L
  VARIANT 93: note = Position 93 is occupied by I, L or V; note (original language) = La posicion 93 esta ocupada por I, L o V
  VARIANT 35: note = Position 35 is occupied by D, E or Q; note (original language) = La posicion 35 esta ocupada por D, E o Q

SEQ ID NO: 46 - protein, 133 aa, synthetic construct; identical to SEQ ID NO: 1
  VARIANT 81: note = Position 81 is occupied by D or E; note (original language) = La posicion 81 esta ocupada por D o E
  VARIANT 83: note = Position 83 is occupied by A, N, G, Q, I, L, M, F, P, S, T, V, W or Y; note (original language) = La posicion 83 esta ocupada por A, N, G, Q, I, L, M, F, P, S, T, V, W o Y
  VARIANT 84: note = Position 84 is occupied by A, N, G, Q, I, L, M, F, P, S, T, V, W or Y; note (original language) = La posicion 84 esta ocupada por A, N, G, Q, I, L, M, F, P, S, T, V, W o Y
  VARIANT 87: note = Position 87 is occupied by D or E; note (original language) = La posicion 87 esta ocupada por D o E
  VARIANT 80: note = Position 80 is occupied by F, I, L, M or V; note (original language) = La posicion 80 esta ocupada por F, I, L, M o V
  VARIANT 82: note = Position 82 is occupied by A or P; note (original language) = La posicion 82 esta ocupada por A o P
  VARIANT 85: note = Position 85 is occupied by I, L, M or V; note (original language) = La posicion 85 esta ocupada por I, L, M or V
  VARIANT 86: note = Position 86 is occupied by I or V; note (original language) = La posicion 86 esta ocupada por I o V
  VARIANT 89: note = Position 89 is occupied by I, L or M; note (original language) = La posicion 89 esta ocupada por I, L o M
  VARIANT 92: note = Position 92 is occupied by I or L; note (original language) = La posicion 92 esta ocupada por I o L
  VARIANT 93: note = Position 93 is occupied by I, L or V; note (original language) = La posicion 93 esta ocupada por I, L o V
  VARIANT 35: note = Position 35 is occupied by D, E or Q; note (original language) = La posicion 35 esta ocupada por D, E o Q

SEQ ID NO: 47 - protein, 133 aa, synthetic construct; identical to SEQ ID NO: 1
  VARIANT 81: note = Position 81 is occupied by A, N, G, Q, I, L, M, F, P, S, T, V, W or Y; note (original language) = La posicion 81 esta ocupada por A, N, G, Q, I, L, M, F, P, S, T, V, W o Y
  VARIANT 83: note = Position 83 is occupied by D or E; note (original language) = La posicion 83 esta ocupada por D o E
  VARIANT 84: note = Position 81 is occupied by A, N, G, Q, I, L, M, F, P, S, T, V, W or Y; note (original language) = La posicion 81 esta ocupada por A, N, G, Q, I, L, M, F, P, S, T, V, W o Y
  VARIANT 87: note = Position 87 is occupied by D or E; note (original language) = La posicion 84 esta ocupada por D o E
  VARIANT 80: note = Position 80 is occupied by F, I, L, M or V; note (original language) = La posicion 80 esta ocupada por F, I, L, M o V
  VARIANT 82: note = Position 82 is occupied by A or P; note (original language) = La posicion 82 esta ocupada por A o P
  VARIANT 85: note = Position 85 is occupied by I, L, M or V; note (original language) = La posicion 85 esta ocupada por I, L, M or V
  VARIANT 86: note = Position 86 is occupied by I or V; note (original language) = La posicion 86 esta ocupada por I o V
  VARIANT 89: note = Position 89 is occupied by I, L or M; note (original language) = La posicion 89 esta ocupada por I, L o M
  VARIANT 92: note = Position 92 is occupied by I or L; note (original language) = La posicion 92 esta ocupada por I o L
  VARIANT 93: note = Position 93 is occupied by I, L or V; note (original language) = La posicion 93 esta ocupada por I, L o V
  VARIANT 35: note = Position 35 is occupied by D, E or Q; note (original language) = La posicion 35 esta ocupada por D, E o Q

SEQ ID NO: 48 - protein, 133 aa, synthetic construct; identical to SEQ ID NO: 1
  VARIANT 81: note = Position 81 is occupied by D or E; note (original language) = La posicion 81 esta ocupada por D o E
  VARIANT 83: note = Position 83 is occupied by A, N, G, Q, I, L, M, F, P, S, T, V, W or Y; note (original language) = La posicion 83 esta ocupada por A, N, G, Q, I, L, M, F, P, S, T, V, W o Y
  VARIANT 84: note = Position 84 is occupied by D or E; note (original language) = La posicion 84 esta ocupada por D o E
  VARIANT 80: note = Position 80 is occupied by F, I, L, M or V; note (original language) = La posicion 80 esta ocupada por F, I, L, M o V
  VARIANT 82: note = Position 82 is occupied by A or P; note (original language) = La posicion 82 esta ocupada por A o P
  VARIANT 85: note = Position 85 is occupied by I, L, M or V; note (original language) = La posicion 85 esta ocupada por I, L, M or V
  VARIANT 86: note = Position 86 is occupied by I or V; note (original language) = La posicion 86 esta ocupada por I o V
  VARIANT 89: note = Position 89 is occupied by I, L or M; note (original language) = La posicion 89 esta ocupada por I, L o M
  VARIANT 92: note = Position 92 is occupied by I or L; note (original language) = La posicion 92 esta ocupada por I o L
  VARIANT 93: note = Position 93 is occupied by I, L or V; note (original language) = La posicion 93 esta ocupada por I, L o V
  VARIANT 35: note = Position 35 is occupied by D, E or Q; note (original language) = La posicion 35 esta ocupada por D, E o Q
  VARIANT 87: note = Position 87 is occupied by D or E; note (original language) = La posicion 87 esta ocupada por D o E

SEQ ID NO: 49 - protein, 133 aa, synthetic construct; identical to SEQ ID NO: 1
  VARIANT 81: note = Position 81 is occupied by A, N, G, Q, I, L, M, F, P, S, T, V, W or Y; note (original language) = La posicion 81 esta ocupada por A, N, G, Q, I, L, M, F, P, S, T, V, W o Y
  VARIANT 83: note = Position 83 is occupied by D or E; note (original language) = La posicion 83 esta ocupada por D o E
  VARIANT 84: note = Position 84 is occupied by D or E; note (original language) = La posicion 84 esta ocupada por D o E
  VARIANT 87: note = Position 87 is occupied by D or E; note (original language) = La posicion 87 esta ocupada por D o E
  VARIANT 80: note = Position 80 is occupied by F, I, L, M or V; note (original language) = La posicion 80 esta ocupada por F, I, L, M o V
  VARIANT 82: note = Position 82 is occupied by A or P; note (original language) = La posicion 82 esta ocupada por A o P
  VARIANT 85: note = Position 85 is occupied by I, L, M or V; note (original language) = La posicion 85 esta ocupada por I, L, M or V
  VARIANT 86: note = Position 86 is occupied by I or V; note (original language) = La posicion 86 esta ocupada por I o V
  VARIANT 89: note = Position 89 is occupied by I, L or M; note (original language) = La posicion 89 esta ocupada por I, L o M
  VARIANT 92: note = Position 92 is occupied by I or L; note (original language) = La posicion 92 esta ocupada por I o L
  VARIANT 93: note = Position 93 is occupied by I, L or V; note (original language) = La posicion 93 esta ocupada por I, L o V
  VARIANT 35: note = Position 35 is occupied by D, E or Q; note (original language) = La posicion 35 esta ocupada por D, E o Q

SEQ ID NO: 50 - protein, 133 aa, synthetic construct; identical to SEQ ID NO: 1
  VARIANT 81: note = Position 81 is occupied by D or E; note (original language) = La posicion 81 esta ocupada por D o E
  VARIANT 83: note = Position 83 is occupied by D or E; note (original language) = La posicion 83 esta ocupada por D o E
  VARIANT 84: note = Position 84 is occupied by D or E; note (original language) = La posicion 84 esta ocupada por D o E
  VARIANT 87: note = Position 87 is occupied by A, N, G, Q, I, L, M, F, P, S, T, V, W or Y; note (original language) = La posicion 87 esta ocupada por A, N, G, Q, I, L, M, F, P, S, T, V, W o Y
  VARIANT 80: note = Position 80 is occupied by F, I, L, M or V; note (original language) = La posicion 80 esta ocupada por F, I, L, M o V
  VARIANT 82: note = Position 82 is occupied by A or P; note (original language) = La posicion 82 esta ocupada por A o P
  VARIANT 85: note = Position 85 is occupied by I, L, M or V; note (original language) = La posicion 85 esta ocupada por I, L, M or V
  VARIANT 86: note = Position 86 is occupied by I or V; note (original language) = La posicion 86 esta ocupada por I o V
  VARIANT 89: note = Position 89 is occupied by I, L or M; note (original language) = La posicion 89 esta ocupada por I, L o M
  VARIANT 92: note = Position 92 is occupied by I or L; note (original language) = La posicion 92 esta ocupada por I o L
  VARIANT 93: note = Position 93 is occupied by I, L or V; note (original language) = La posicion 93 esta ocupada por I, L o V
  VARIANT 35: note = Position 35 is occupied by D, E or Q; note (original language) = La posicion 35 esta ocupada por D, E o Q

SEQ ID NO: 51 - protein, 133 aa, synthetic construct; identical to SEQ ID NO: 1
  VARIANT 81: note = Position 81 is occupied by D or E; note (original language) = La posicion 81 esta ocupada por D o E
  VARIANT 83: note = Position 84 is occupied by D or E; note (original language) = La posicion 83 esta ocupada por D o E
  VARIANT 84: note = Position 84 is occupied by A, N, G, Q, I, L, M, F, P, S, T, V, W or Y; note (original language) = La posicion 84 esta ocupada por A, N, G, Q, I, L, M, F, P, S, T, V, W o Y
  VARIANT 87: note = Position 87 is occupied by D or E; note (original language) = La posicion 87 esta ocupada por D o E
  VARIANT 80: note = Position 80 is occupied by F, I, L, M or V; note (original language) = La posicion 80 esta ocupada por F, I, L, M o V
  VARIANT 82: note = Position 82 is occupied by A or P; note (original language) = La posicion 82 esta ocupada por A o P
  VARIANT 85: note = Position 85 is occupied by I, L, M or V; note (original language) = La posicion 85 esta ocupada por I, L, M or V
  VARIANT 86: note = Position 86 is occupied by I or V; note (original language) = La posicion 86 esta ocupada por I o V
  VARIANT 89: note = Position 89 is occupied by I, L or M; note (original language) = La posicion 89 esta ocupada por I, L o M
  VARIANT 92: note = Position 92 is occupied by I or L; note (original language) = La posicion 92 esta ocupada por I o L
  VARIANT 93: note = Position 93 is occupied by I, L or V; note (original language) = La posicion 93 esta ocupada por I, L o V; note = Position 35 is occupied by D, E or Q; note (original language) = La posicion 35 esta ocupada por K, D, E o Q

SEQ ID NO: 52 - protein, 133 aa, synthetic construct; identical to SEQ ID NO: 1
  VARIANT 81: note = Position 81 is occupied by D or E; note (original language) = La posicion 81 esta ocupada por D o E
  VARIANT 83: note = Position 83 is occupied by D or E; note (original language) = La posicion 83 esta ocupada por D o E
  VARIANT 84: note = Position 84 is occupied by D or E; note (original language) = La posicion 84 esta ocupada por D o E
  VARIANT 87: note = Position 87 is occupied by D or E; note (original language) = La posicion 87 esta ocupada por D o E
  VARIANT 80: note = Position 80 is occupied by F, I, L, M or V; note (original language) = La posicion 80 esta ocupada por F, I, L, M o V
  VARIANT 82: note = Position 82 is occupied by A or P; note (original language) = La posicion 82 esta ocupada por A o P
  VARIANT 85: note = Position 85 is occupied by I, L, M or V; note (original language) = La posicion 85 esta ocupada por I, L, M or V
  VARIANT 86: note = Position 86 is occupied by I or V; note (original language) = La posicion 86 esta ocupada por I o V
  VARIANT 89: note = Position 89 is occupied by I, L or M; note (original language) = La posicion 89 esta ocupada por I, L o M
  VARIANT 92: note = Position 92 is occupied by I or L; note (original language) = La posicion 92 esta ocupada por I o L
  VARIANT 93: note = Position 93 is occupied by I, L or V; note (original language) = La posicion 93 esta ocupada por I, L o V
  VARIANT 35: note = Position 35 is occupied by D, E or Q; note (original language) = La posicion 35 esta ocupada por D, E o Q

SEQ ID NO: 53 - protein, 133 aa, synthetic construct
APTSSSTKKTQLQLEHLLLDLQMILNGINNYKNPKLTRMLTFKFYMPKKATELKHLQCLEEELKPLEEVLNLAQSKNFHLDPQDLIDNINVIVLELKGSETTFMCEYADETATIVEFLNRWITFSQSIISTLT

SEQ ID NO: 54 - protein, 133 aa, synthetic construct
APTSSSTKKTQLQLEHLLLDLQMILNGINNYKNPKLTRMLTFKFYMPKKATELKHLQCLEEELKPLEEVLNLAQSKNFHLVPADLIENINVIVLELKGSETTFMCEYADETATIVEFLNRWITFSQSIISTLT

SEQ ID NO: 55 - protein, 133 aa, synthetic construct
APTSSSTKKTQLQLEHLLLDLQMILNGINNYKNPKLTRMLTFKFYMPKKATELKHLQCLEEELKPLEEVLNLAQSKNFHLDPSDLIENINVIVLELKGSETTFMCEYADETATIVEFLNRWITFSQSIISTLT

SEQ ID NO: 56 - protein, 133 aa, synthetic construct
APTSSSTKKTQLQLEHLLLDLQMILNGINNYKNPKLTRMLTFKFYMPKKATELKHLQCLEEELKPLEEVLNLAQSKNFHLVPAELITNINVIVLELKGSETTFMCEYADETATIVEFLNRWITFSQSIISTLT

SEQ ID NO: 57 - protein, 133 aa, synthetic construct
APTSSSTKKTQLQLEHLLLDLQMILNGINNYKNPKLTRMLTFKFYMPKKATELKHLQCLEEELKPLEEVLNLAQSKNFHLAPPELIENINVIVLELKGSETTFMCEYADETATIVEFLNRWITFSQSIISTLT

SEQ ID NO: 58 - protein, 133 aa, synthetic construct
APTSSSTKKTQLQLEHLLLDLQMILNGINNYKNPKLTRMLTFKFYMPKKATELKHLQCLEEELKPLEEVLNLAQSKNFHLAAVGLIQNINVIVLELKGSETTFMCEYADETATIVEFLNRWITFSQSIISTLT

SEQ ID NO: 59 - protein, 133 aa, synthetic construct
APTSSSTKKTQLQLEHLLLDLQMILNGINNYKNPKLTRMLTFKFYMPKKATELKHLQCLEEELKPLEEVLNLAQSKNFHLPAEELIENINVIVLELKGSETTFMCEYADETATIVEFLNRWITFSQSIISTLT

SEQ ID NO: 60 - protein, 133 aa, synthetic construct
APTSSSTKKTQLQLEHLLLDLQMILNGINNYKNPKLTRMLTFKFYMPKKATELKHLQCLEEELKPLEEVLNLAQSKNFHLSPLDLIDNINVIVLELKGSETTFMCEYADETATIVEFLNRWITFSQSIISTLT

SEQ ID NO: 61 - protein, 133 aa, synthetic construct
APTSSSTKKTQLQLEHLLLDLQMILNGINNYKNPKLTRMLTFKFYMPKKATELKHLQCLEEELKPLEEVLNLAQSKNFHLVPTDLIDNINVIVLELKGSETTFMCEYADETATIVEFLNRWITFSQSIISTLT

SEQ ID NO: 62 - protein, 133 aa, synthetic construct
APTSSSTKKTQLQLEHLLLDLQMILNGINNYKNPKLTRMLTFKFYMPKKATELKHLQCLEEELKPLEEVLNLAQSKNFHLSAVQLISNINVIVLELKGSETTFMCEYADETATIVEFLNRWITFSQSIISTLT

SEQ ID NO: 63 - protein, 133 aa, synthetic construct
APTSSSTKKTQLQLEHLLLDLQMILNGINNYKNPKLTRMLTFKFYMPKKATELKHLQCLEEELKPLEEVLNLAQSKNFHLLAQDLIDNINVIVLELKGSETTFMCEYADETATIVEFLNRWITFSQSIISTLT

SEQ ID NO: 64 - protein, 133 aa, synthetic construct
APTSSSTKKTQLQLEHLLLDLQMILNGINNYKNPKLTRMLTFKFYMPKKATELKHLQCLEEELKPLEEVLNLAQSKNFHLIAQDLIDNINVIVLELKGSETTFMCEYADETATIVEFLNRWITFSQSIISTLT

SEQ ID NO: 65 - protein, 133 aa, synthetic construct
APTSSSTKKTQLQLEHLLLDLQMILNGINNYKNPKLTRMLTFKFYMPKKATELKHLQCLEEELKPLEEVLNLAQSKNFHLTPEELIENINVIVLELKGSETTFMCEYADETATIVEFLNRWITFSQSIISTLT

SEQ ID NO: 66 - protein, 133 aa, synthetic construct
APTSSSTKKTQLQLEHLLLDLQMILNGINNYKNPKLTRMLTFKFYMPKKATELKHLQCLEEELKPLEEVLNLAQSKNFHLVPEDLIQNINVIVLELKGSETTFMCEYADETATIVEFLNRWITFSQSIISTLT

SEQ ID NO: 67 - protein, 133 aa, synthetic construct
APTSSSTKKTQLQLEHLLLDLQMILNGINNYKNPKLTRMLTFKFYMPKKATELKHLQCLEEELKPLEEVLNLAQSKNFHLDPQLLIENINVIVLELKGSETTFMCEYADETATIVEFLNRWITFSQSIISTLT

SEQ ID NO: 68 - protein, 133 aa, synthetic construct
APTSSSTKKTQLQLEHLLLDLQMILNGINNYKNPKLTRMLTFKFYMPKKATELKHLQCLEEELKPLEEVLNLAQSKNFHLDPAELIENINVIVLELKGSETTFMCEYADETATIVEFLNRWITFSQSIISTLT

SEQ ID NO: 69 - protein, 133 aa, synthetic construct
APTSSSTKKTQLQLEHLLLDLQMILNGINNYKNPKLTRMLTFKFYMPKKATELKHLQCLEEELKPLEEVLNLAQSKNFHLDPNELIENINVIVLELKGSETTFMCEYADETATIVEFLNRWITFSQSIISTLT

SEQ ID NO: 70 - protein, 133 aa, synthetic construct
APTSSSTKKTQLQLEHLLLDLQMILNGINNYKNPKLTRMLTFKFYMPKKATELKHLQCLEEELKPLEEVLNLAQSKNFHLAPSDLIENINVIVLELKGSETTFMCEYADETATIVEFLNRWITFSQSIISTLT

SEQ ID NO: 71 - protein, 133 aa, synthetic construct
APTSSSTKKTQLQLEHLLLDLQMILNGINNYKNPKLTRMLTFKFYMPKKATELKHLQCLEEELKPLEEVLNLAQSKNFHLDPADLIQNINVIVLELKGSETTFMCEYADETATIVEFLNRWITFSQSIISTLT

SEQ ID NO: 72 - protein, 133 aa, synthetic construct
APTSSSTKKTQLQLEHLLLDLQMILNGINNYKNPKLTRMLTFKFYMPKKATELKHLQCLEEELKPLEEVLNLAQSKNFHLKPDELIENINLIVLELKGSETTFMCEYADETATIVEFLNRWITFSQSIISTLT

SEQ ID NO: 73 - protein, 133 aa, synthetic construct
APTSSSTKKTQLQLEHLLLDLQMILNGINNYKNPKLTRMLTFKFYMPKKATELKHLQCLEEELKPLEEVLNLAQSKNFHLAPEELIDNINVIVLELKGSETTFMCEYADETATIVEFLNRWITFSQSIISTLT

SEQ ID NO: 74 - protein, 133 aa, synthetic construct
APTSSSTKKTQLQLEHLLLDLQMILNGINNYKNPKLTRMLTFKFYMPKKATELKHLQCLEEELKPLEEVLNLAQSKNFHLTPPELIENINVIVLELKGSETTFMCEYADETATIVEFLNRWITFSQSIISTLT

SEQ ID NO: 75 - protein, 133 aa, synthetic construct
APTSSSTKKTQLQLEHLLLDLQMILNGINNYKNPKLTRMLTFKFYMPKKATELKHLQCLEEELKPLEEVLNLAQSKNFHLRPEELIENINVIVLELKGSETTFMCEYADETATIVEFLNRWITFSQSIISTLT

SEQ ID NO: 76 - protein, 133 aa, synthetic construct
APTSSSTKKTQLQLEHLLLDLQMILNGINNYKNPKLTRMLTFKFYMPKKATELKHLQCLEEELKPLEEVLNLAQSKNFHLLPSELIENINVIVLELKGSETTFMCEYADETATIVEFLNRWITFSQSIISTLT

SEQ ID NO: 77 - protein, 133 aa, synthetic construct
APTSSSTKKTQLQLEHLLLDLQMILNGINNYKNPKLTRMLTFKFYMPKKATELKHLQCLEEELKPLEEVLNLAQSKNFHLVPEELIENINVIVLELKGSETTFMCEYADETATIVEFLNRWITFSQSIISTLT

SEQ ID NO: 78 - protein, 133 aa, synthetic construct
APTSSSTKKTQLQLEHLLLDLQMILNGINNYKNPKLTRMLTFKFYMPKKATELKHLQCLEEELKPLEEVLNLAQSKNFHLDPQELIDNINVIVLELKGSETTFMCEYADETATIVEFLNRWITFSQSIISTLT

SEQ ID NO: 79 - protein, 133 aa, synthetic construct
APTSSSTKKTQLQLEHLLLDLQMILNGINNYKNPKLTRMLTFKFYMPKKATELKHLQCLEEELKPLEEVLNLAQSKNFHLVPEDLIDNINVIVLELKGSETTFMCEYADETATIVEFLNRWITFSQSIISTLT

SEQ ID NO: 80 - protein, 133 aa, synthetic construct
APTSSSTKKTQLQLEHLLLDLQMILNGINNYKNPKLTRMLTFKFYMPKKATELKHLQCLEEELKPLEEVLNLAQSKNFHLNAQELIENINVIVLELKGSETTFMCEYADETATIVEFLNRWITFSQSIISTLT

SEQ ID NO: 81 - protein, 133 aa, synthetic construct
APTSSSTKKTQLQLEHLLLDLQMILNGINNYKNPKLTRMLTFKFYMPKKATELKHLQCLEEELKPLEEVLNLAQSKNFHLDAQDLISNINVIVLELKGSETTFMCEYADETATIVEFLNRWITFSQSIISTLT

SEQ ID NO: 82 - protein, 133 aa, synthetic construct
APTSSSTKKTQLQLEHLLLDLQMILNGINNYKNPKLTRMLTFKFYMPKKATELKHLQCLEEELKPLEEVLNLAQSKNFHLVPAELIENINVIVLELKGSETTFMCEYADETATIVEFLNRWITFSQSIISTLT

SEQ ID NO: 83 - protein, 133 aa, synthetic construct
APTSSSTKKTQLQLEHLLLDLQMILNGINNYKNPKLTRMLTFKFYMPKKATELKHLQCLEEELKPLEEVLNLAQSKNFHLAPQDLIENINVIVLELKGSETTFMCEYADETATIVEFLNRWITFSQSIISTLT

SEQ ID NO: 84 - protein, 133 aa, synthetic construct
APTSSSTKKTQLQLEHLLLDLQMILNGINNYKNPKLTRMLTFKFYMPKKATELKHLQCLEEELKPLEEVLNLAQSKNFHLPPSDLIENINVIVLELKGSETTFMCEYADETATIVEFLNRWITFSQSIISTLT

SEQ ID NO: 85 - protein, 133 aa, synthetic construct
APTSSSTKKTQLQLEHLLLDLQMILNGINNYKNPKLTRMLTFKFYMPKKATELKHLQCLEEELKPLEEVLNLAQSKNFHLEADVLIENINVIVLELKGSETTFMCEYADETATIVEFLNRWITFSQSIISTLT

SEQ ID NO: 86 - protein, 133 aa, synthetic construct
APTSSSTKKTQLQLEHLLLDLQMILNGINNYKNPKLTRMLTFKFYMPKKATELKHLQCLEEELKPLEEVLNLAQSKNFHMAPSDLIENINVIVLELKGSETTFMCEYADETATIVEFLNRWITFSQSIISTLT

SEQ ID NO: 87 - protein, 133 aa, synthetic construct
APTSSSTKKTQLQLEHLLLDLQMILNGINNYKNPKLTRMLTFKFYMPKKATELKHLQCLEEELKPLEEVLNLAQSKNFHLSPSELIENINVIVLELKGSETTFMCEYADETATIVEFLNRWITFSQSIISTLT

SEQ ID NO: 88 - protein, 133 aa, synthetic construct
APTSSSTKKTQLQLEHLLLDLQMILNGINNYKNPKLTRMLTFKFYMPKKATELKHLQCLEEELKPLEEVLNLAQSKNFHLEPAELIENINVIVLELKGSETTFMCEYADETATIVEFLNRWITFSQSIISTLT

SEQ ID NO: 89 - protein, 133 aa, synthetic construct
APTSSSTKKTQLQLEHLLLDLQMILNGINNYKNPKLTRMLTFKFYMPKKATELKHLQCLEEELKPLEEVLNLAQSKNFHLSPQELIENINVIVLELKGSETTFMCEYADETATIVEFLNRWITFSQSIISTLT

SEQ ID NO: 90 - protein, 133 aa, synthetic construct
APTSSSTKKTQLQLEHLLLDLQMILNGINNYKNPKLTRMLTFKFYMPKKATELKHLQCLEEELKPLEEVLNLAQSKNFHLVPSDLIENINVIVLELKGSETTFMCEYADETATIVEFLNRWITFSQSIISTLT

SEQ ID NO: 91 - protein, 133 aa, synthetic construct
APTSSSTKKTQLQLEHLLLDLQMILNGINNYKNPKLTRMLTFKFYMPKKATELKHLQCLEEELKPLEEVLNLAQSKNFHLPARDLIENINVIVLELKGSETTFMCEYADETATIVEFLNRWITFSQSIISTLT

SEQ ID NO: 92 - protein, 133 aa, synthetic construct
APTSSSTKKTQLQLEHLLLDLQMILNGINNYKNPKLTRMLTFKFYMPKKATELKHLQCLEEELKPLEEVLNLAQSKNFHLTPQDLIDNINVIVLELKGSETTFMCEYADETATIVEFLNRWITFSQSIISTLT

SEQ ID NO: 93 - protein, 133 aa, synthetic construct
APTSSSTKKTQLQLEHLLLDLQMILNGINNYKNPKLTRMLTFKFYMPKKATELKHLQCLEEELKPLEEVLNLAQSKNFHLVPQELIENINVIVLELKGSETTFMCEYADETATIVEFLNRWITFSQSIISTLT

SEQ ID NO: 94 - protein, 133 aa, synthetic construct
APTSSSTKKTQLQLEHLLLDLQMILNGINNYKNPKLTRMLTFKFYMPKKATELKHLQCLEEELKPLEEVLNLAQSKNFHLQPQELIENINVIVLELKGSETTFMCEYADETATIVEFLNRWITFSQSIISTLT

SEQ ID NO: 95 - protein, 133 aa, synthetic construct; identical to SEQ ID NO: 90

SEQ ID NO: 96 - protein, 133 aa, synthetic construct
APTSSSTKKTQLQLEHLLLDLQMILNGINNYKNPKLTRMLTFKFYMPKKATELKHLQCLEEELKPLEEVLNLAQSKNFHLDPSELIENINVIVLELKGSETTFMCEYADETATIVEFLNRWITFSQSIISTLT

SEQ ID NO: 97 - protein, 133 aa, synthetic construct
APTSSSTKKTQLQLEHLLLDLQMILNGINNYKNPKLTRMLTFKFYMPKKATELKHLQCLEEELKPLEEVLNLAQSKNFHLDAATLIENINVIVLELKGSETTFMCEYADETATIVEFLNRWITFSQSIISTLT

SEQ ID NO: 98 - protein, 133 aa, synthetic construct
APTSSSTKKTQLQLEHLLLDLQMILNGINNYKNPKLTRMLTFKFYMPKKATELKHLQCLEEELKPLEEVLNLAQSKNFHLDAKDLIENINVIVLELKGSETTFMCEYADETATIVEFLNRWITFSQSIISTLT

SEQ ID NO: 99 - protein, 133 aa, synthetic construct
APTSSSTKKTQLQLEHLLLDLQMILNGINNYKNPKLTRMLTFKFYMPKKATELKHLQCLEEELKPLEEVLNLAQSKNFHLQPQDLIENINVIVLELKGSETTFMCEYADETATIVEFLNRWITFSQSIISTLT

SEQ ID NO: 100 - protein, 133 aa, synthetic construct
APTSSSTKKTQLQLEHLLLDLQMILNGINNYKNPKLTRMLTFKFYMPKKATELKHLQCLEEELKPLEEVLNLAQSKNFHLPPDDLIENINVIVLELKGSETTFMCEYADETATIVEFLNRWITFSQSIISTLT

SEQ ID NO: 101 - protein, 133 aa, synthetic construct
APTSSSTKKTQLQLEHLLLDLQMILNGINNYKNPKLTRMLTFKFYMPKKATELKHLQCLEEELKPLEEVLNLAQSKNFHFDPHDVVENINVLLLELKGSETTFMCEYADETATIVEFLNRWITFSQSIISTLT

SEQ ID NO: 102 - protein, 133 aa, synthetic construct
APTSSSTKKTQLQLEHLLLDLQMILNGINNYKNPKLTRMLTFKFYMPKKATELKHLQCLEEELKPLEEVLNLAQSKNFHVPPEDLIANINVLVLELKGSETTFMCEYADETATIVEFLNRWITFSQSIISTLT

SEQ ID NO: 103 - protein, 133 aa, synthetic construct
APTSSSTKKTQLQLEHLLLDLQMILNGINNYKNPKLTRMLTFKFYMPKKATELKHLQCLEEELKPLEEVLNLAQSKNFHLTPADVVDNMNVLILELKGSETTFMCEYADETATIVEFLNRWITFSQSIISTLT

SEQ ID NO: 104 - protein, 133 aa, synthetic construct
APTSSSTKKTQLQLEHLLLDLQMILNGINNYKNPKLTRMLTFKFYMPKKATELKHLQCLEEELKPLEEVLNLAQSKNFHMSPADMIDNMNVLILELKGSETTFMCEYADETATIVEFLNRWITFSQSIISTLT

SEQ ID NO: 105 - protein, 133 aa, synthetic construct
APTSSSTKKTQLQLEHLLLDLQMILNGINNYKNPKLTRMLTFKFYMPKKATELKHLQCLEEELKPLEEVLNLAQSKNFHIEPAEVIQNINVLVLELKGSETTFMCEYADETATIVEFLNRWITFSQSIISTLT

SEQ ID NO: 106 - protein, 133 aa, synthetic construct
APTSSSTKKTQLQLEHLLLDLQMILNGINNYKNPKLTRMLTFKFYMPKKATELKHLQCLEEELKPLEEVLNLAQSKNFHFDPSDVVANMNVILLELKGSETTFMCEYADETATIVEFLNRWITFSQSIISTLT

SEQ ID NO: 107 - protein, 133 aa, synthetic construct
APTSSSTKKTQLQLEHLLLDLQMILNGINNYKNPKLTRMLTFKFYMPKKATELKHLQCLEEELKPLEEVLNLAQSKNFHLEPDEVVSNLNVLILELKGSETTFMCEYADETATIVEFLNRWITFSQSIISTLT

SEQ ID NO: 108 - protein, 133 aa, synthetic construct
APTSSSTKKTQLQLEHLLLDLQMILNGINNYKNPKLTRMLTFKFYMPKKATELKHLQCLEEELKPLEEVLNLAQSKNFHLDAAELIDNLNVLILELKGSETTFMCEYADETATIVEFLNRWITFSQSIISTLT

SEQ ID NO: 109 - protein, 133 aa, synthetic construct
APTSSSTKKTQLQLEHLLLDLQMILNGINNYKNPKLTRMLTFKFYMPKKATELKHLQCLEEELKPLEEVLNLAQSKNFHMSPEDIISNLNVLVLELKGSETTFMCEYADETATIVEFLNRWITFSQSIISTLT

SEQ ID NO: 110 - protein, 133 aa, synthetic construct
APTSSSTKKTQLQLEHLLLDLQMILNGINNYKNPKLTRMLTFKFYMPKKATELKHLQCLEEELKPLEEVLNLAQSKNFHMTAGDVIENINVLLLELKGSETTFMCEYADETATIVEFLNRWITFSQSIISTLT

SEQ ID NO: 111 - protein, 133 aa, synthetic construct
APTSSSTKKTQLQLEHLLLDLQMILNGINNYKNPKLTRMLTFKFYMPKKATELKHLQCLEEELKPLEEVLNLAQSKNFHLVPEELIDNMNVLLLELKGSETTFMCEYADETATIVEFLNRWITFSQSIISTLT

SEQ ID NO: 112 - protein, 133 aa, synthetic construct
APTSSSTKKTQLQLEHLLLDLQMILNGINNYKNPKLTRMLTFKFYMPKKATELKHLQCLEEELKPLEEVLNLAQSKNFHINPEDLIENLNVLLLELKGSETTFMCEYADETATIVEFLNRWITFSQSIISTLT

SEQ ID NO: 113 - protein, 229 aa, synthetic construct
ASDKTHTCPPCPAPELLGGPSVFLFPPKPKDTLMISRTPEVTCVVVDVSHEDPEVKFNWYVDGVEVHNAKTKPREEQYNSTYRVVSVLTVLHQDWLNGKEYKCKVSNKALPAPIEKTISKAKGQPREPQVYTLPPSREEVTKNQVSLTCLVKGFYPSDIAVEWESNGQPENNYKTTPPVLDSDGSFFLYSKLTVDKSRWQQGNVFSCSVMHEALHNHYTQKSLSLSPGK

SEQ ID NO: 114 - protein, 133 aa, synthetic construct
APTSSSTKKTQLQLEHLLLDLQMILNGINNYKNPELTRMLTFKFYMPKKATELKHLQCLEEELKPLEEVLNLAQSKNFHLDPQDLIENINVIVLELKGSETTFMCEYADETATIVEFLNRWITFSQSIISTLT

SEQ ID NO: 115 - protein, 133 aa, synthetic construct
APTSSSTKKTQLQLEHLLLDLQMILNGINNYKNPELTRMLTFKFYMPKKATELKHLQCLEEELKPLEEVLNLAQSKNFHLVPEDLIENINVIVLELKGSETTFMCEYADETATIVEFLNRWITFSQSIISTLT

SEQ ID NO: 116 - protein, 133 aa, synthetic construct
APTSSSTKKTQLQLEHLLLDLQMILNGINNYKNPELTRMLTFKFYMPKKATELKHLQCLEEELKPLEEVLNLAQSKNFHLDPQDLIENINVLVLELKGSETTFMCEYADETATIVEFLNRWITFSQSIISTLT

SEQ ID NO: 117 - protein, 133 aa, synthetic construct
APTSSSTKKTQLQLEHLLLDLQMILNGINNYKNPELTRMLTFKFYMPKKATELKHLQCLEEELKPLEEVLNLAQSKNFHLVPEDLIENINVLVLELKGSETTFMCEYADETATIVEFLNRWITFSQSIISTLT

SEQ ID NO: 118 - protein, 133 aa, synthetic construct
APTSSSTKKTQLQLEHLLLDLQMILNGINNYKNPELTRMLTFKFYMPKKATELKHLQCLEEELKPLEEVLNLAQSKNFHFDPHDVVENINVLLLELKGSETTFMCEYADETATIVEFLNRWITFSQSIISTLT

SEQ ID NO: 119 - protein, 133 aa, synthetic construct
APTSSSTKKTQLQLEHLLLDLQMILNGINNYKNPELTRMLTFKFYMPKKATELKHLQCLEEELKPLEEVLNLAQSKNFHVPPEDLIANINVLVLELKGSETTFMCEYADETATIVEFLNRWITFSQSIISTLT

SEQ ID NO: 120 - protein, 133 aa, synthetic construct
APTSSSTKKTQLQLEHLLLDLQMILNGINNYKNPELTRMLTFKFYMPKKATELKHLQCLEEELKPLEEVLNLAQSKNFHVPPEDLIENINVLVLELKGSETTFMCEYADETATIVEFLNRWITFSQSIISTLT

SEQ ID NO: 121 - protein, 133 aa, synthetic construct
APTSSSTKKTQLQLEHLLLDLQMILNGINNYKNPELTRMLTFKFYMPKKATELKHLQCLEEELKPLEEVLNLAQSKNFHFDPADVVENINVLVLELKGSETTFMCEYADETATIVEFLNRWITFSQSIISTLT

SEQ ID NO: 122 - protein, 133 aa, synthetic construct
APTSSSTKKTQLQLEHLLLDLQMILNGINNYKNPELTRMLTFKFYMPKKATELKHLQCLEEELKPLEEVLNLAQSKNFHFDPEDVVENINVLVLELKGSETTFMCEYADETATIVEFLNRWITFSQSIISTLT

SEQ ID NO: 123 - protein, 229 aa, synthetic construct
ASDKTHTCPPCPAPEAAGGPSVFLFPPKPKDTLMISRTPEVTCVVVDVSHEDPEVKFNWYVDGVEVHNAKTKPREEQYNSTYRVVSVLTVLHQDWLNGKEYKCKVSNKALPAPIEKTISKAKGQPREPQVYTLPPSREEVTKNQVSLTCLVKGFYPSDIAVEWESNGQPENNYKTTPPVLDSDGSFFLYSKLTVDKSRWQQGNVFSCSVMHEALHNHYTQKSLSLSPGK

SEQ ID NO: 124 - protein, 133 aa, synthetic construct
APTSSSTKKTQLQLEHLLLDLQMILNGINNYKNPELTAMLTAKFAMPKKATELKHLQCLEEALKPLEEVLNLAQSKNFHVPPEDLIENINVLVLELKGSETTFMCEYADETATIVEFLNRWITFSQSIISTLT

SEQ ID NO: 125 - protein, 133 aa, synthetic construct
APTSSSTKKTQLQLEHLLLDLQMILNGINNYKNPELTRMLTFKFYMPKKATELKHLQCLEEELKPLEEVLNLAQSKNFHFDPADVVENINVFVLELKGSETTFMCEYADETATIVEFLNRWITFSQSIISTLT

SEQ ID NO: 126 - protein, 133 aa, synthetic construct
APTSSSTKKTQLQLEHLLLDLQMILNGINNYKNPELTRMLTFKFYMPKKATELKHLQCLEEELKPLEEVLNLAQSKNFHFDPEDVVENINVFVLELKGSETTFMCEYADETATIVEFLNRWITFSQSIISTLT

SEQ ID NO: 127 - protein, 133 aa, synthetic construct; identical to SEQ ID NO: 27
  VARIANT 81: note = Position 81 is occupied by H,K or R; note (original language) = La posicion 81 esta ocupada por H,K o R
  VARIANT 83: note = Position 83 is occupied by D or E; note (original language) = La posicion 83 esta ocupada por D o E
  VARIANT 84: note = Position 84 is occupied by D or E; note (original language) = La posicion 84 esta ocupada por D o E
  VARIANT 87: note = Position 87 is occupied by D or E; note (original language) = La posicion 87 esta ocupada por D o E
  VARIANT 92: note = Position 92 is occupied by I or L; note (original language) = La posicion 92 esta ocupada por I o L
  VARIANT 35: note = Position 35 is occupied by K, D, E or Q; note (original language) = La posicion 35 esta ocupada por K, D, E o Q

SEQ ID NO: 128 - protein, 133 aa, synthetic construct; identical to SEQ ID NO: 27
  VARIANT 81: note = Position 81 is occupied by D or E; note (original language) = La posicion 81 esta ocupada por D o E
  VARIANT 83: note = Position 83 is occupied by H, K or R; note (original language) = La posicion 83 esta ocupada por H, K o R
  VARIANT 84: note = Position 84 is occupied by D or E; note (original language) = La posicion 84 esta ocupada por D o E
  VARIANT 87: note = Position 87 is occupied by D or E; note (original language) = La posicion 87 esta ocupada por D o E
  VARIANT 92: note = Position 92 is occupied by I or L; note (original language) = La posicion 92 esta ocupada por I o L
  VARIANT 35: note = Position 35 is occupied by K, D, E or Q; note (original language) = La posicion 35 esta ocupada por K, D, E o Q

SEQ ID NO: 129 - protein, 133 aa, synthetic construct; identical to SEQ ID NO: 27
  VARIANT 81: note = Position 81 is occupied by A, N, G, Q, I, L, M, F, P, S, T, V, W or Y; note (original language) = La posicion 81 esta ocupada por A, N, G, Q, I, L, M, F, P, S, T, V, W o Y
  VARIANT 83: note = Position 83 is occupied by A, N, G, Q, I, L, M, F, P, S, T, V, W or Y; note (original language) = La posicion 83 esta ocupada por A, N, G, Q, I, L, M, F, P, S, T, V, W o Y
  VARIANT 84: note = Position 84 is occupied by D or E; note (original language) = La posicion 84 esta ocupada por D o E
  VARIANT 87: note = Position 87 is occupied by D or E; note (original language) = La posicion 87 esta ocupada por D o E
  VARIANT 92: note = Position 92 is occupied by I or L; note (original language) = La posicion 92 esta ocupada por I o L
  VARIANT 35: note = Position 35 is occupied by K, D, E or Q; note (original language) = La posicion 35 esta ocupada por K, D, E o Q; note = Position 35 is occupied by K, D, E or Q; note (original language) = La posicion 35 esta ocupada por K, D, E o Q

SEQ ID NO: 130 - protein, 133 aa, synthetic construct; identical to SEQ ID NO: 27
  VARIANT 81: note = Position 81 is occupied by D or E; note (original language) = La posicion 81 esta ocupada por D o E
  VARIANT 83: note = Position 83 is occupied by A, N, G, Q, I, L, M, F, P, S, T, V, W or Y; note (original language) = La posicion 83 esta ocupada por A, N, G, Q, I, L, M, F, P, S, T, V, W o Y
  VARIANT 84: note = Position 84 is occupied by D or E; note (original language) = La posicion 84 esta ocupada por D o E
  VARIANT 87: note = Position 87 is occupied by A, N, G, Q, I, L, M, F, P, S, T, V, W or Y; note (original language) = La posicion 87 esta ocupada por A, N, G, Q, I, L, M, F, P, S, T, V, W o Y
  VARIANT 92: note = Position 92 is occupied by I or L; note (original language) = La posicion 92 esta ocupada por I o L
  VARIANT 35: note = Position 35 is occupied by K, D, E or Q; note (original language) = La posicion 35 esta ocupada por K, D, E o Q

SEQ ID NO: 131 - protein, 133 aa, synthetic construct; identical to SEQ ID NO: 27
  VARIANT 81: note = Position 81 is occupied by A, N, G, Q, I, L, M, F, P, S, T, V, W or Y; note (original language) = La posicion 81 esta ocupada por A, N, G, Q, I, L, M, F, P, S, T, V, W o Y
  VARIANT 83: note = Position 83 is occupied by D or E; note (original language) = La posicion 83 esta ocupada por D o E
  VARIANT 84: note = Position 84 is occupied by D or E; note (original language) = La posicion 84 esta ocupada por D o E
  VARIANT 87: note = Position 87 is occupied by A, N, G, Q, I, L, M, F, P, S, T, V, W or Y; note (original language) = La posicion 87 esta ocupada por A, N, G, Q, I, L, M, F, P, S, T, V, W o Y
  VARIANT 92: note = Position 92 is occupied by I or L; note (original language) = La posicion 92 esta ocupada por I o L
  VARIANT 35: note = Position 35 is occupied by K, D, E or Q; note (original language) = La posicion 35 esta ocupada por K, D, E o Q

SEQ ID NO: 132 - protein, 133 aa, synthetic construct; identical to SEQ ID NO: 27
  VARIANT 81: note = Position 81 is occupied by D or E; note (original language) = La posicion 81 esta ocupada por D o E
  VARIANT 83: note = Position 83 is occupied by D or E; note (original language) = La posicion 83 esta ocupada por D o E
  VARIANT 84: note = Position 84 is occupied by A, N, G, Q, I, L, M, F, P, S, T, V, W or Y; note (original language) = La posicion 84 esta ocupada por A, N, G, Q, I, L, M, F, P, S, T, V, W o Y
  VARIANT 87: note = Position 87 is occupied by A, N, G, Q, I, L, M, F, P, S, T, V, W or Y; note (original language) = La posicion 87 esta ocupada por A, N, G, Q, I, L, M, F, P, S, T, V, W o Y
  VARIANT 92: note = Position 92 is occupied by I or L; note (original language) = La posicion 92 esta ocupada por I o L
  VARIANT 35: note = Position 35 is occupied by K, D, E or Q; note (original language) = La posicion 35 esta ocupada por K, D, E o Q

SEQ ID NO: 133 - protein, 133 aa, synthetic construct; identical to SEQ ID NO: 27
  VARIANT 81: note = Position 81 is occupied by D or E; note (original language) = La posicion 81 esta ocupada por D o E
  VARIANT 83: note = Position 83 is occupied by A, N, G, Q, I, L, M, F, P, S, T, V, W or Y; note (original language) = La posicion 83 esta ocupada por A, N, G, Q, I, L, M, F, P, S, T, V, W o Y
  VARIANT 84: note = Position 84is occupied by A, N, G, Q, I, L, M, F, P, S, T, V, W or Y; note (original language) = La posicion 84 esta ocupada por A, N, G, Q, I, L, M, F, P, S, T, V, W o Y
  VARIANT 87: note = Position 87 is occupied by D or E; note (original language) = La posicion 87 esta ocupada por D o E
  VARIANT 92: note = Position 92 is occupied by I or L; note (original language) = La posicion 92 esta ocupada por I o L
  VARIANT 35: note = Position 35 is occupied by K, D, E or Q; note (original language) = La posicion 35 esta ocupada por K, D, E o Q

SEQ ID NO: 134 - protein, 133 aa, synthetic construct; identical to SEQ ID NO: 27
  VARIANT 81: note = Position 81 is occupied by A, N, G, Q, I, L, M, F, P, S, T, V, W or Y; note (original language) = La posicion 81 esta ocupada por A, N, G, Q, I, L, M, F, P, S, T, V, W o Y
  VARIANT 83: note = Position 83 is occupied by D or E; note (original language) = La posicion 83 esta ocupada por D o E
  VARIANT 84: note = Position 84 is occupied by A, N, G, Q, I, L, M, F, P, S, T, V, W or Y; note (original language) = La posicion 84 esta ocupada por A, N, G, Q, I, L, M, F, P, S, T, V, W o Y
  VARIANT 87: note = Position 87 is occupied by D or E; note (original language) = La posicion 87 esta ocupada por D o E
  VARIANT 92: note = Position 92 is occupied by I or L; note (original language) = La posicion 92 esta ocupada por I o L
  VARIANT 35: note = Position 35 is occupied by K, D, E or Q; note (original language) = La posicion 35 esta ocupada por K, D, E o Q

SEQ ID NO: 135 - protein, 133 aa, synthetic construct; identical to SEQ ID NO: 27
  VARIANT 81: note = Position 81 is occupied by D or E; note (original language) = La posicion 81 esta ocupada por D o E
  VARIANT 83: note = Position 83 is occupied by A, N, G, Q, I, L, M, F, P, S, T, V, W or Y; note (original language) = La posicion 83 esta ocupada por A, N, G, Q, I, L, M, F, P, S, T, V, W o Y
  VARIANT 84: note = Position 84 is occupied by D or E; note (original language) = La posicion 84 esta ocupada por D o E
  VARIANT 87: note = Position 87 is occupied by D or E; note (original language) = La posicion 87 esta ocupada por D o E
  VARIANT 92: note = Position 92 is occupied by I or L; note (original language) = La posicion 92 esta ocupada por I o L
  VARIANT 35: note = Position 35 is occupied by K, D, E or Q; note (original language) = La posicion 35 esta ocupada por K, D, E o Q

SEQ ID NO: 136 - protein, 133 aa, synthetic construct; identical to SEQ ID NO: 27
  VARIANT 81: note = Position 81 is occupied by A, N, G, Q, I, L, M, F, P, S, T, V, W or Y; note (original language) = La posicion 81 esta ocupada por A, N, G, Q, I, L, M, F, P, S, T, V, W o Y
  VARIANT 83: note = Position 83 is occupied by D or E; note (original language) = La posicion 83 esta ocupada por D o E
  VARIANT 84: note = Position 84 is occupied by D or E; note (original language) = La posicion 84 esta ocupada por D o E
  VARIANT 87: note = Position 87 is occupied by D or E; note (original language) = La posicion 87 esta ocupada por D o E
  VARIANT 92: note = Position 92 is occupied by I or L; note (original language) = La posicion 92 esta ocupada por I o L
  VARIANT 35: note = Position 35 is occupied by K, D, E or Q; note (original language) = La posicion 35 esta ocupada por K, D, E o Q

SEQ ID NO: 137 - protein, 133 aa, synthetic construct; identical to SEQ ID NO: 27
  VARIANT 81: note = Position 81 is occupied by D or E; note (original language) = La posicion 81 esta ocupada por D o E
  VARIANT 83: note = Position 83 is occupied by D or E; note (original language) = La posicion 83 esta ocupada por D o E
  VARIANT 84: note = Position 84 is occupied by D or E; note (original language) = La posicion 84 esta ocupada por D o E
  VARIANT 87: note = Position 87 is occupied by A, N, G, Q, I, L, M, F, P, S, T, V, W or Y; note (original language) = La posicion 87 esta ocupada por A, N, G, Q, I, L, M, F, P, S, T, V, W o Y
  VARIANT 35: note = Position 35 is occupied by K, D, E or Q; note (original language) = La posicion 35 esta ocupada por K, D, E o Q

SEQ ID NO: 138 - protein, 133 aa, synthetic construct; identical to SEQ ID NO: 27
  VARIANT 81: note = Position 81 is occupied by D or E; note (original language) = La posicion 81 esta ocupada por D o E
  VARIANT 83: note = Position 83 is occupied by D or E; note (original language) = La posicion 83 esta ocupada por D o E
  VARIANT 84: note = Position 84 is occupied by A, N, G, Q, I, L, M, F, P, S, T, V, W or Y; note (original language) = La posicion 84 esta ocupada por A, N, G, Q, I, L, M, F, P, S, T, V, W o Y
  VARIANT 87: note = Position 87 is occupied by D or E; note (original language) = La posicion 87 esta ocupada por D o E
  VARIANT 92: note = Position 92 is occupied by I or L; note (original language) = La posicion 92 esta ocupada por I o L
  VARIANT 35: note = Position 35 is occupied by K, D, E or Q; note (original language) = La posicion 35 esta ocupada por K, D, E o Q

SEQ ID NO: 139 - protein, 133 aa, synthetic construct; identical to SEQ ID NO: 27
  VARIANT 81: note = Position 81 is occupied by D or E; note (original language) = La posicion 81 esta ocupada por D o E
  VARIANT 83: note = Position 83 is occupied by D or E; note (original language) = La posicion 83 esta ocupada por D o E
  VARIANT 84: note = Position 84 is occupied by D or E; note (original language) = La posicion 84 esta ocupada por D o E
  VARIANT 87: note = Position 87 is occupied by D or E; note (original language) = La posicion 87 esta ocupada por D o E
  VARIANT 92: note = Position 92 is occupied by I or L; note (original language) = La posicion 92 esta ocupada por I o L
  VARIANT 35: note = Position 35 is occupied by K, D, E or Q; note (original language) = La posicion 35 esta ocupada por K, D, E o Q

SEQ ID NO: 140 - protein, 133 aa, unidentified; identical to SEQ ID NO: 27
  VARIANT 81: note = Position 81 is occupied by H, K or R; note (original language) = La posicion 81 esta ocupada por H, K o R
  VARIANT 83: note = Position 83 is occupied by D or E; note (original language) = La posicion 83 esta ocupada por D o E
  VARIANT 84: note = Position 84 is occupied by D or E; note (original language) = La posicion 84 esta ocupada por D o E
  VARIANT 87: note = Position 87 is occupied by D or E; note (original language) = La posicion 87 esta ocupada por D o E
  VARIANT 80: note = Position 80 is occupied by F, I, L, M or V; note (original language) = La posicion 80 esta ocupada por F, I, L, M o V
  VARIANT 82: note = Position 82 is occupied by A or P; note (original language) = La posicion 82 esta ocupada por A o P
  VARIANT 85: note = Position 85 is occupied by I, L, M or V; note (original language) = La posicion 85 esta ocupada por I, L, M or V
  VARIANT 86: note = Position 86 is occupied by I or V; note (original language) = La posicion 86 esta ocupada por I o V
  VARIANT 89: note = Position 89 is occupied by I, L or M; note (original language) = La posicion 89 esta ocupada por I, L o M
  VARIANT 92: note = Position 92 is occupied by I or L; note (original language) = La posicion 92 esta ocupada por I o L
  VARIANT 93: note = Position 93 is occupied by I, L or V; note (original language) = La posicion 93 esta ocupada por I, L o V
  VARIANT 35: note = Position 35 is occupied by K, D, E or Q; note (original language) = La posicion 35 esta ocupada por K, D, E o Q

SEQ ID NO: 141 - protein, 133 aa, synthetic construct; identical to SEQ ID NO: 27
  VARIANT 81: note = Position 81 is occupied by D or E; note (original language) = La posicion 81 esta ocupada por D o E
  VARIANT 83: note = Position 83 is occupied by H, K or R; note (original language) = La posicion 83 esta ocupada por H, K o R
  VARIANT 84: note = Position 84 is occupied by D or E; note (original language) = La posicion 84 esta ocupada por D o E
  VARIANT 87: note = Position 87 is occupied by D or E; note (original language) = La posicion 87 esta ocupada por D o E
  VARIANT 80: note = Position 80 is occupied by F, I, L, M or V; note (original language) = La posicion 80 esta ocupada por F, I, L, M o V
  VARIANT 82: note = Position 82 is occupied by A or P; note (original language) = La posicion 82 esta ocupada por A o P
  VARIANT 85: note = Position 85 is occupied by I, L, M or V; note (original language) = La posicion 85 esta ocupada por I, L, M or V
  VARIANT 86: note = Position 86 is occupied by I or V; note (original language) = La posicion 86 esta ocupada por I o V
  VARIANT 89: note = Position 89 is occupied by I, L or M; note (original language) = La posicion 89 esta ocupada por I, L o M
  VARIANT 92: note = Position 92 is occupied by I or L; note (original language) = La posicion 92 esta ocupada por I o L
  VARIANT 93: note = Position 93 is occupied by I, L or V; note (original language) = La posicion 93 esta ocupada por I, L o V
  VARIANT 35: note = Position 35 is occupied by K, D, E or Q; note (original language) = La posicion 35 esta ocupada por K, D, E o Q

SEQ ID NO: 142 - protein, 133 aa, synthetic construct; identical to SEQ ID NO: 27
  VARIANT 81: note = Position 81 is occupied by A, N, G, Q, I, L, M, F, P, S, T, V, W or Y; note (original language) = La posicion 81 esta ocupada por A, N, G, Q, I, L, M, F, P, S, T, V, W o Y
  VARIANT 83: note = Position 83 is occupied by A, N, G, Q, I, L, M, F, P, S, T, V, W or Y; note (original language) = La posicion 83 esta ocupada por A, N, G, Q, I, L, M, F, P, S, T, V, W o Y
  VARIANT 84: note = Position 84 is occupied by D or E; note (original language) = La posicion 84 esta ocupada por D o E
  VARIANT 87: note = Position 87 is occupied by D or E; note (original language) = La posicion 87 esta ocupada por D o E
  VARIANT 80: note = Position 80 is occupied by F, I, L, M or V; note (original language) = La posicion 80 esta ocupada por F, I, L, M o V
  VARIANT 82: note = Position 82 is occupied by A or P; note (original language) = La posicion 82 esta ocupada por A o P
  VARIANT 85: note = Position 85 is occupied by I, L, M or V; note (original language) = La posicion 85 esta ocupada por I, L, M or V
  VARIANT 86: note = Position 86 is occupied by I or V; note (original language) = La posicion 86 esta ocupada por I o V
  VARIANT 89: note = Position 89 is occupied by I, L or M; note (original language) = La posicion 89 esta ocupada por I, L o M
  VARIANT 92: note = Position 92 is occupied by I or L; note (original language) = La posicion 92 esta ocupada por I o L
  VARIANT 93: note = Position 93 is occupied by I, L or V; note (original language) = La posicion 93 esta ocupada por I, L o V
  VARIANT 35: note = Position 35 is occupied by K, D, E or Q; note (original language) = La posicion 35 esta ocupada por K, D, E o Q

SEQ ID NO: 143 - protein, 133 aa, synthetic construct; identical to SEQ ID NO: 27
  VARIANT 81: note = Position 81 is occupied by D or E; note (original language) = La posicion 81 esta ocupada por D o E
  VARIANT 83: note = Position 83 is occupied by A, N, G, Q, I, L, M, F, P, S, T, V, W or Y; note (original language) = La posicion 83 esta ocupada por A, N, G, Q, I, L, M, F, P, S, T, V, W o Y
  VARIANT 84: note = Position 84 is occupied by D or E; note (original language) = La posicion 84 esta ocupada por D o E
  VARIANT 87: note = Position 87 is occupied by A, N, G, Q, I, L, M, F, P, S, T, V, W or Y; note (original language) = La posicion 87 esta ocupada por A, N, G, Q, I, L, M, F, P, S, T, V, W o Y
  VARIANT 80: note = Position 80 is occupied by F, I, L, M or V; note (original language) = La posicion 80 esta ocupada por F, I, L, M o V
  VARIANT 82: note = Position 82 is occupied by A or P; note (original language) = La posicion 82 esta ocupada por A o P
  VARIANT 85: note = Position 85 is occupied by I, L, M or V; note (original language) = La posicion 85 esta ocupada por I, L, M or V
  VARIANT 86: note = Position 86 is occupied by I or V; note (original language) = La posicion 86 esta ocupada por I o V
  VARIANT 89: note = Position 89 is occupied by I, L or M; note (original language) = La posicion 89 esta ocupada por I, L o M
  VARIANT 92: note = Position 92 is occupied by I or L; note (original language) = La posicion 92 esta ocupada por I o L
  VARIANT 93: note = Position 93 is occupied by I, L or V; note (original language) = La posicion 93 esta ocupada por I, L o V
  VARIANT 35: note = Position 35 is occupied by K, D, E or Q; note (original language) = La posicion 35 esta ocupada por K, D, E o Q

SEQ ID NO: 144 - protein, 133 aa, synthetic construct; identical to SEQ ID NO: 27
  VARIANT 81: note = Position 81 is occupied by A, N, G, Q, I, L, M, F, P, S, T, V, W or Y; note (original language) = La posicion 81 esta ocupada por A, N, G, Q, I, L, M, F, P, S, T, V, W o Y
  VARIANT 83: note = Position 83 is occupied by D or E; note (original language) = La posicion 83 esta ocupada por D o E
  VARIANT 84: note = Position 84 is occupied by D or E; note (original language) = La posicion 84 esta ocupada por D o E
  VARIANT 87: note = Position 87 is occupied by A, N, G, Q, I, L, M, F, P, S, T, V, W or Y; note (original language) = La posicion 87 esta ocupada por A, N, G, Q, I, L, M, F, P, S, T, V, W o Y
  VARIANT 80: note = Position 80 is occupied by F, I, L, M or V; note (original language) = La posicion 80 esta ocupada por F, I, L, M o V
  VARIANT 82: note = Position 82 is occupied by A or P; note (original language) = La posicion 82 esta ocupada por A o P
  VARIANT 85: note = Position 85 is occupied by I, L, M or V; note (original language) = La posicion 85 esta ocupada por I, L, M or V
  VARIANT 86: note = Position 86 is occupied by I or V; note (original language) = La posicion 86 esta ocupada por I o V
  VARIANT 89: note = Position 89 is occupied by I, L or M; note (original language) = La posicion 89 esta ocupada por I, L o M
  VARIANT 92: note = Position 92 is occupied by I or L; note (original language) = La posicion 92 esta ocupada por I o L
  VARIANT 93: note = Position 93 is occupied by I, L or V; note (original language) = La posicion 93 esta ocupada por I, L o V
  VARIANT 35: note = Position 35 is occupied by K, D, E or Q; note (original language) = La posicion 35 esta ocupada por K, D, E o Q

SEQ ID NO: 145 - protein, 133 aa, synthetic construct; identical to SEQ ID NO: 27
  VARIANT 81: note = Position 81 is occupied by D or E; note (original language) = La posicion 81 esta ocupada por D o E
  VARIANT 83: note = Position 83 is occupied by D or E; note (original language) = La posicion 83 esta ocupada por D o E
  VARIANT 84: note = Position 84 is occupied by A, N, G, Q, I, L, M, F, P, S, T, V, W or Y; note (original language) = La posicion 84 esta ocupada por A, N, G, Q, I, L, M, F, P, S, T, V, W o Y
  VARIANT 87: note = Position 87 is occupied by A, N, G, Q, I, L, M, F, P, S, T, V, W or Y; note (original language) = La posicion 87 esta ocupada por A, N, G, Q, I, L, M, F, P, S, T, V, W o Y
  VARIANT 80: note = Position 80 is occupied by F, I, L, M or V; note (original language) = La posicion 80 esta ocupada por F, I, L, M o V
  VARIANT 82: note = Position 82 is occupied by A or P; note (original language) = La posicion 82 esta ocupada por A o P
  VARIANT 85: note = Position 85 is occupied by I, L, M or V; note (original language) = La posicion 85 esta ocupada por I, L, M or V
  VARIANT 86: note = Position 86 is occupied by I or V; note (original language) = La posicion 86 esta ocupada por I o V
  VARIANT 89: note = Position 89 is occupied by I, L or M; note (original language) = La posicion 89 esta ocupada por I, L o M
  VARIANT 92: note = Position 92 is occupied by I or L; note (original language) = La posicion 92 esta ocupada por I o L
  VARIANT 93: note = Position 93 is occupied by I, L or V; note (original language) = La posicion 93 esta ocupada por I, L o V
  VARIANT 35: note = Position 35 is occupied by K, D, E or Q; note (original language) = La posicion 35 esta ocupada por K, D, E o Q

SEQ ID NO: 146 - protein, 133 aa, synthetic construct; identical to SEQ ID NO: 27
  VARIANT 81: note = Position 81 is occupied by D or E; note (original language) = La posicion 81 esta ocupada por D o E
  VARIANT 83: note = Position 83 is occupied by A, N, G, Q, I, L, M, F, P, S, T, V, W or Y; note (original language) = La posicion 83 esta ocupada por A, N, G, Q, I, L, M, F, P, S, T, V, W o Y
  VARIANT 84: note = Position 84 is occupied by A, N, G, Q, I, L, M, F, P, S, T, V, W or Y; note (original language) = La posicion 84 esta ocupada por A, N, G, Q, I, L, M, F, P, S, T, V, W o Y
  VARIANT 87: note = Position 87 is occupied by D or E; note (original language) = La posicion 87 esta ocupada por D o E
  VARIANT 80: note = Position 80 is occupied by F, I, L, M or V; note (original language) = La posicion 80 esta ocupada por F, I, L, M o V
  VARIANT 82: note = Position 82 is occupied by A or P; note (original language) = La posicion 82 esta ocupada por A o P
  VARIANT 85: note = Position 85 is occupied by I, L, M or V; note (original language) = La posicion 85 esta ocupada por I, L, M or V
  VARIANT 86: note = Position 86 is occupied by I or V; note (original language) = La posicion 86 esta ocupada por I o V
  VARIANT 89: note = Position 89 is occupied by I, L or M; note (original language) = La posicion 89 esta ocupada por I, L o M
  VARIANT 92: note = Position 92 is occupied by I or L; note (original language) = La posicion 92 esta ocupada por I o L
  VARIANT 93: note = Position 93 is occupied by I, L or V; note (original language) = La posicion 93 esta ocupada por I, L o V
  VARIANT 35: note = Position 35 is occupied by K, D, E or Q; note (original language) = La posicion 35 esta ocupada por K, D, E o Q

SEQ ID NO: 147 - protein, 133 aa, synthetic construct; identical to SEQ ID NO: 27
  VARIANT 81: note = Position 81 is occupied by A, N, G, Q, I, L, M, F, P, S, T, V, W or Y; note (original language) = La posicion 81 esta ocupada por A, N, G, Q, I, L, M, F, P, S, T, V, W o Y
  VARIANT 83: note = Position 83 is occupied by D or E; note (original language) = La posicion 83 esta ocupada por D o E
  VARIANT 84: note = Position 84 is occupied by A, N, G, Q, I, L, M, F, P, S, T, V, W or Y; note (original language) = La posicion 84 esta ocupada por A, N, G, Q, I, L, M, F, P, S, T, V, W o Y
  VARIANT 87: note = Position 87 is occupied by D or E; note (original language) = La posicion 87 esta ocupada por D o E
  VARIANT 80: note = Position 80 is occupied by F, I, L, M or V; note (original language) = La posicion 80 esta ocupada por F, I, L, M o V
  VARIANT 82: note = Position 82 is occupied by A or P; note (original language) = La posicion 82 esta ocupada por A o P
  VARIANT 85: note = Position 85 is occupied by I, L, M or V; note (original language) = La posicion 85 esta ocupada por I, L, M or V
  VARIANT 86: note = Position 86 is occupied by I or V; note (original language) = La posicion 86 esta ocupada por I o V
  VARIANT 89: note = Position 89 is occupied by I, L or M; note (original language) = La posicion 89 esta ocupada por I, L o M
  VARIANT 92: note = Position 92 is occupied by I or L; note (original language) = La posicion 92 esta ocupada por I o L
  VARIANT 93: note = Position 93 is occupied by I, L or V; note (original language) = La posicion 93 esta ocupada por I, L o V
  VARIANT 35: note = Position 35 is occupied by K, D, E or Q; note (original language) = La posicion 35 esta ocupada por K, D, E o Q

SEQ ID NO: 148 - protein, 133 aa, synthetic construct; identical to SEQ ID NO: 27
  VARIANT 81: note = Position 81 is occupied by D or E; note (original language) = La posicion 81 esta ocupada por D o E
  VARIANT 83: note = Position 83 is occupied by A, N, G, Q, I, L, M, F, P, S, T, V, W or Y; note (original language) = La posicion 83 esta ocupada por A, N, G, Q, I, L, M, F, P, S, T, V, W o Y
  VARIANT 84: note = Position 84 is occupied by D or E; note (original language) = La posicion 84 esta ocupada por D o E
  VARIANT 87: note = Position 87 is occupied by D or E; note (original language) = La posicion 87 esta ocupada por D o E
  VARIANT 80: note = Position 80 is occupied by F, I, L, M or V; note (original language) = La posicion 80 esta ocupada por F, I, L, M o V
  VARIANT 82: note = Position 82 is occupied by A or P; note (original language) = La posicion 82 esta ocupada por A o P
  VARIANT 85: note = Position 85 is occupied by I, L, M or V; note (original language) = La posicion 85 esta ocupada por I, L, M or V
  VARIANT 86: note = Position 86 is occupied by I or V; note (original language) = La posicion 86 esta ocupada por I o V
  VARIANT 89: note = Position 89 is occupied by I, L or M; note (original language) = La posicion 89 esta ocupada por I, L o M
  VARIANT 92: note = Position 92 is occupied by I or L; note (original language) = La posicion 92 esta ocupada por I o L
  VARIANT 93: note = Position 93 is occupied by I, L or V; note (original language) = La posicion 93 esta ocupada por I, L o V
  VARIANT 35: note = Position 35 is occupied by K, D, E or Q; note (original language) = La posicion 35 esta ocupada por K, D, E o Q

SEQ ID NO: 149 - protein, 133 aa, synthetic construct; identical to SEQ ID NO: 27
  VARIANT 81: note = Position 81 is occupied by A, N, G, Q, I, L, M, F, P, S, T, V, W or Y; note (original language) = La posicion 81 esta ocupada por A, N, G, Q, I, L, M, F, P, S, T, V, W o Y
  VARIANT 83: note = Position 83 is occupied by D or E; note (original language) = La posicion 83 esta ocupada por D o E
  VARIANT 84: note = Position 84 is occupied by D or E; note (original language) = La posicion 84 esta ocupada por D o E
  VARIANT 87: note = Position 87 is occupied by D or E; note (original language) = La posicion 87 esta ocupada por D o E
  VARIANT 80: note = Position 80 is occupied by F, I, L, M or V; note (original language) = La posicion 80 esta ocupada por F, I, L, M o V
  VARIANT 82: note = Position 82 is occupied by A or P; note (original language) = La posicion 82 esta ocupada por A o P
  VARIANT 85: note = Position 85 is occupied by I, L, M or V; note (original language) = La posicion 85 esta ocupada por I, L, M or V
  VARIANT 86: note = Position 86 is occupied by I or V; note (original language) = La posicion 86 esta ocupada por I o V
  VARIANT 89: note = Position 89 is occupied by I, L or M; note (original language) = La posicion 89 esta ocupada por I, L o M
  VARIANT 92: note = Position 92 is occupied by I or L; note (original language) = La posicion 92 esta ocupada por I o L
  VARIANT 93: note = Position 93 is occupied by I, L or V; note (original language) = La posicion 93 esta ocupada por I, L o V
  VARIANT 35: note = Position 35 is occupied by K, D, E or Q; note (original language) = La posicion 35 esta ocupada por K, D, E o Q

SEQ ID NO: 150 - protein, 133 aa, synthetic construct; identical to SEQ ID NO: 27
  VARIANT 81: note = Position 81 is occupied by D or E; note (original language) = La posicion 81 esta ocupada por D o E
  VARIANT 83: note = Position 83 is occupied by D or E; note (original language) = La posicion 83 esta ocupada por D o E
  VARIANT 84: note = Position 84 is occupied by D or E; note (original language) = La posicion 84 esta ocupada por D o E
  VARIANT 87: note = Position 87 is occupied by A, N, G, Q, I, L, M, F, P, S, T, V, W or Y; note (original language) = La posicion 87 esta ocupada por A, N, G, Q, I, L, M, F, P, S, T, V, W o Y
  VARIANT 80: note = Position 80 is occupied by F, I, L, M or V; note (original language) = La posicion 80 esta ocupada por F, I, L, M o V
  VARIANT 82: note = Position 82 is occupied by A or P; note (original language) = La posicion 82 esta ocupada por A o P
  VARIANT 85: note = Position 85 is occupied by I, L, M or V; note (original language) = La posicion 85 esta ocupada por I, L, M or V
  VARIANT 86: note = Position 86 is occupied by I or V; note (original language) = La posicion 86 esta ocupada por I o V
  VARIANT 89: note = Position 89 is occupied by I, L or M; note (original language) = La posicion 89 esta ocupada por I, L o M
  VARIANT 92: note = Position 92 is occupied by I or L; note (original language) = La posicion 92 esta ocupada por I o L
  VARIANT 93: note = Position 93 is occupied by I, L or V; note (original language) = La posicion 93 esta ocupada por I, L o V
  VARIANT 35: note = Position 35 is occupied by K, D, E or Q; note (original language) = La posicion 35 esta ocupada por K, D, E o Q

SEQ ID NO: 151 - protein, 133 aa, synthetic construct; identical to SEQ ID NO: 27
  VARIANT 81: note = Position 81 is occupied by D or E; note (original language) = La posicion 81 esta ocupada por D o E
  VARIANT 83: note = Position 83 is occupied by D or E; note (original language) = La posicion 83 esta ocupada por D o E
  VARIANT 84: note = Position 84 is occupied by A, N, G, Q, I, L, M, F, P, S, T, V, W or Y; note (original language) = La posicion 84 esta ocupada por A, N, G, Q, I, L, M, F, P, S, T, V, W o Y
  VARIANT 87: note = Position 87 is occupied by D or E; note (original language) = La posicion 87 esta ocupada por D o E
  VARIANT 80: note = Position 80 is occupied by F, I, L, M or V; note (original language) = La posicion 80 esta ocupada por F, I, L, M o V
  VARIANT 82: note = Position 82 is occupied by A or P; note (original language) = La posicion 82 esta ocupada por A o P
  VARIANT 85: note = Position 85 is occupied by I, L, M or V; note (original language) = La posicion 85 esta ocupada por I, L, M or V
  VARIANT 86: note = Position 86 is occupied by I or V; note (original language) = La posicion 86 esta ocupada por I o V
  VARIANT 89: note = Position 89 is occupied by I, L or M; note (original language) = La posicion 89 esta ocupada por I, L o M
  VARIANT 92: note = Position 92 is occupied by I or L; note (original language) = La posicion 92 esta ocupada por I o L
  VARIANT 93: note = Position 93 is occupied by I, L or V; note (original language) = La posicion 93 esta ocupada por I, L o V
  VARIANT 35: note = Position 35 is occupied by K, D, E or Q; note (original language) = La posicion 35 esta ocupada por K, D, E o Q

SEQ ID NO: 152 - protein, 133 aa, synthetic construct; identical to SEQ ID NO: 27
  VARIANT 81: note = Position 81 is occupied by D or E; note (original language) = La posicion 81 esta ocupada por D o E
  VARIANT 83: note = Position 83 is occupied by D or E; note (original language) = La posicion 83 esta ocupada por D o E
  VARIANT 84: note = Position 84 is occupied by D or E; note (original language) = La posicion 84 esta ocupada por D o E
  VARIANT 87: note = Position 87 is occupied by D or E; note (original language) = La posicion 87 esta ocupada por D o E
  VARIANT 80: note = Position 80 is occupied by F, I, L, M or V; note (original language) = La posicion 80 esta ocupada por F, I, L, M o V
  VARIANT 82: note = Position 82 is occupied by A or P; note (original language) = La posicion 82 esta ocupada por A o P
  VARIANT 85: note = Position 85 is occupied by I, L, M or V; note (original language) = La posicion 85 esta ocupada por I, L, M or V
  VARIANT 86: note = Position 86 is occupied by I or V; note (original language) = La posicion 86 esta ocupada por I o V
  VARIANT 89: note = Position 89 is occupied by I, L or M; note (original language) = La posicion 89 esta ocupada por I, L o M
  VARIANT 92: note = Position 92 is occupied by I or L; note (original language) = La posicion 92 esta ocupada por I o L
  VARIANT 93: note = Position 93 is occupied by I, L or V; note (original language) = La posicion 93 esta ocupada por I, L o V
  VARIANT 35: note = Position 35 is occupied by K, D, E or Q; note (original language) = La posicion 35 esta ocupada por K, D, E o Q